European Patent Specification EP 3 397 645 B1, published March 25, 2026. Title: VARIABLE REGIONS FOR NKp46 BINDING PROTEINS. Applicant: INNATE PHARMA. The sequence listing filed with the application follows.

SEQUENCE LISTING (218 sequences)

SEQ ID NO: 1 - protein, 304 aa, homo sapiens
MSSTLPALLCVGLCLSQRISAQQQTLPKPFIWAEPHFMVPKEKQVTICCQGNYGAVEYQLHFEGSLFAVDRPKPPERINKVKFYIPDMNSRMAGQYSCIYRVGELWSEPSNLLDLVVTEMYDTPTLSVHPGPEVISGEKVTFYCRLDTATSMFLLLKEGRSSHVQRGYGKVQAEFPLGPVTTAHRGTYRCFGSYNNHAWSFPSEPVKLLVTGDIENTSLAPEDPTFPADTWGTYLLTTETGLQKDHALWDHTAQNLLRMGLAFLVLVALVWFLVEDWLSRKRTRERASRASTWEGRRRLNTQTL

SEQ ID NO: 2 - protein, 216 aa, homo sapiens
APELLGGPSVFLFPPKPKDTLMISRTPEVTCVVVDVSHEDPEVKFNWYVDGVEVHNAKTKPREEQYNSTYRVVSVLTVLHQDWLNGKEYKCKVSNKALPAPIEKTISKAKGQPREPQVYTLPPSREEMTKNQVSLTCLVKGFYPSDIAVEWESNGQPENNYKTTPPVLDSDGSFFLTSKLTVDKSRWQQGNVFSCSVMHEALHNHYTQKSLSLSPG

SEQ ID NO: 3 - protein, 120 aa, Mus musculus
QVQLQQSGPELVKPGASVKMSCKASGYTFTDYVINWGKQRSGQGLEWIGEIYPGSGTNYYNEKFKAKATLTADKSSNIAYMQLSSLTSEDSAVYFCARRGRYGLYAMDYWGQGTSVTVSS

SEQ ID NO: 4 - protein, 107 aa, Mus musculus
DIQMTQTTSSLSASLGDRVTISCRASQDISNYLNWYQQKPDGTVKLLIYYTSRLHSGVPSRFSGSGSGTDYSLTINNLEQEDIATYFCQQGNTRPWTFGGGTKLEIK

SEQ ID NO: 5 - protein, 122 aa, Mus musculus
EVQLQESGPGLVKPSQSLSLTCTVTGYSITSDYAWNWIRQFPGNKLEWMGYITYSGSTSYNPSLESRISITRDTSTNQFFLQLNSVTTEDTATYYCARGGYYGSSWGVFAYWGQGTLVTVSA

SEQ ID NO: 6 - protein, 107 aa, Mus musculus
DIQMTQSPASLSASVGETVTITCRVSENIYSYLAWYQQKQGKSPQLLVYNAKTLAEGVPSRFSGSGSGTQFSLKINSLQPEDFGSYYCQHHYGTPWTFGGGTKLEIK

SEQ ID NO: 7 - protein, 116 aa, Mus musculus
EVQLQQSGPELVKPGASVKISCKTSGYTFTEYTMHWVKQSHGKSLEWIGGISPNIGGTSYNQKFKGKATLTVDKSSSTAYMELRSLTSEDSAVYYCARRGGSFDYWGQGTTLTVSS

SEQ ID NO: 8 - protein, 107 aa, Mus musculus
DIVMTQSPATLSVTPGDRVSLSCRASQSISDYLHWYQQKSHESPRLLIKYASQSISGIPSRFSGSGSGSDFTLSINSVEPEDVGVYYCQNGHSFPLTFGAGTKLELK

SEQ ID NO: 9 - protein, 117 aa, Mus musculus
QVQLQQSAVELARPGASVKMSCKASGYTFTSFTMHWVKQRPGQGLEWIGYINPSSGYTEYNQKFKDKTTLTADKSSSTAYMQLDSLTSDDSAVYYCVRGSSRGFDYWGQGTLVTVSA

SEQ ID NO: 10 - protein, 107 aa, Mus musculus
DIQMIQSPASLSVSVGETVTITCRASENIYSNLAWFQQKQGKSPQLLVYAATNLADGVPSRFSGSGSGTQYSLKINSLQSEDFGIYYCQHFWGTPRTFGGGTKLEIK

SEQ ID NO: 11 - protein, 115 aa, Mus musculus
QVQLQQPGSVLVRPGASVKLSCKASGYTFTSSWMHWAKQRPGQGLEWIGHIHPNSGISNYNEKFKGKATLTVDTSSSTAYVDLSSLTSEDSAVYYCARGGRFDDWGAGTTVTVSS

SEQ ID NO: 12 - protein, 107 aa, Mus musculus
DIQMTQSPSSLSASLGERVSLTCRASQDIGSSLNWLQQEPDGTIKRLIYATSSLDSGVPKRFSGSRSGSDYSLTISSLESEDFVDYYCLQYASSPWTFGGGTKLEIK

SEQ ID NO: 13 - protein, 120 aa, Mus musculus
DVQLQESGPGLVKPSQSLSLTCTVTGYSITSDYAWNWIRQFPGNKLEWMGYITYSGSTNYNPSLKSRISITRDTSKNQFFLQLNSVTTEDTATYYCARCWDYALYAMDCWGQGTSVTVSS

SEQ ID NO: 14 - protein, 107 aa, Mus musculus
DIQMTQSPASLSASVGETVTITCRTSENIYSYLAWCQQKQGKSPQLLVYNAKTLAEGVPSRFSGSGSGTHFSLKINSLQPEDFGIYYCQHHYDTPLTFGAGTKLELK

SEQ ID NO: 15 - protein, 5 aa, mus musculus
DYVIN

SEQ ID NO: 16 - protein, 7 aa, mus musculus
GYTFTDY

SEQ ID NO: 17 - protein, 8 aa, mus musculus
GYTFTDYV

SEQ ID NO: 18 - protein, 17 aa, mus musculus
EIYPGSGTNYYNEKFKA

SEQ ID NO: 19 - protein, 4 aa, mus musculus
PGSG

SEQ ID NO: 20 - protein, 16 aa, mus musculus
GYTFTDYVIYPGSGTN

SEQ ID NO: 21 - protein, 11 aa, mus musculus
RGRYGLYAMDY

SEQ ID NO: 22 - protein, 9 aa, mus musculus
GRYGLYAMD

SEQ ID NO: 23 - protein, 13 aa, mus musculus
ARRGRYGLYAMDY

SEQ ID NO: 24 - protein, 11 aa, mus musculus
RASQDISNYLN

SEQ ID NO: 25 - protein, 7 aa, Mus musculus
SQDISNY

SEQ ID NO: 26 - protein, 6 aa, mus musculus
QDISNY

SEQ ID NO: 27 - protein, 7 aa, Mus musculus
YTSRLHS

SEQ ID NO: 28 - protein, 9 aa, mus musculus
QQGNTRPWT

SEQ ID NO: 29 - protein, 9 aa, Mus musculus
YTSGNTRPW

SEQ ID NO: 30 - protein, 12 aa, Mus musculus
YTSQQGNTRPWT

SEQ ID NO: 31 - protein, 6 aa, Mus musculus
SDYAWN

SEQ ID NO: 32 - protein, 8 aa, Mus musculus
GYSITSDY

SEQ ID NO: 33 - protein, 9 aa, Mus musculus
GYSITSDYA

SEQ ID NO: 34 - protein, 16 aa, Mus musculus
YITYSGSTSYNPSLES

SEQ ID NO: 35 - protein, 7 aa, Mus musculus
ITYSGST

SEQ ID NO: 36 - protein, 13 aa, Mus musculus
GGYYGSSWGVFAY

SEQ ID NO: 37 - protein, 11 aa, Mus musculus
GYYGSSWGVFA

SEQ ID NO: 38 - protein, 15 aa, Mus musculus
ARGGYYGSSWGVFAY

SEQ ID NO: 39 - protein, 11 aa, Mus musculus
RVSENIYSYLA

SEQ ID NO: 40 - protein, 7 aa, Mus musculus
SENIYSY

SEQ ID NO: 41 - protein, 6 aa, Mus musculus
ENIYSY

SEQ ID NO: 42 - protein, 7 aa, Mus musculus
NAKTLAE

SEQ ID NO: 43 - protein, 9 aa, Mus musculus
QHHYGTPWT

SEQ ID NO: 44 - protein, 6 aa, Mus musculus
HYGTPW

SEQ ID NO: 45 - protein, 9 aa, mus musculus
QHHYGTPWT

SEQ ID NO: 46 - protein, 5 aa, Mus musculus
EYTMH

SEQ ID NO: 47 - protein, 7 aa, Mus musculus
GYTFTEY

SEQ ID NO: 48 - protein, 8 aa, Mus musculus
GYTFTEYT

SEQ ID NO: 49 - protein, 17 aa, Mus musculus
GISPNIGGTSYNQKFKG

SEQ ID NO: 50 - protein, 8 aa, Mus musculus
ISPNIGGT

SEQ ID NO: 51 - protein, 7 aa, Mus musculus
RGGSFDY

SEQ ID NO: 52 - protein, 5 aa, Mus musculus
GGSFD

SEQ ID NO: 53 - protein, 9 aa, Mus musculus
ARRGGSFDY

SEQ ID NO: 54 - protein, 11 aa, Mus musculus
RASQSISDYLH

SEQ ID NO: 55 - protein, 7 aa, Mus musculus
SQSISDY

SEQ ID NO: 56 - protein, 6 aa, Mus musculus
QSISDY

SEQ ID NO: 57 - protein, 7 aa, Mus musculus
YASQSIS

SEQ ID NO: 58 - protein, 9 aa, Mus musculus
QNGHSFPLT

SEQ ID NO: 59 - protein, 6 aa, Mus musculus
GHSFPL

SEQ ID NO: 60 - protein, 5 aa, Mus musculus
SFTMH

SEQ ID NO: 61 - protein, 7 aa, Mus musculus
GYTFTSF

SEQ ID NO: 62 - protein, 8 aa, Mus musculus
GYTFTSFT

SEQ ID NO: 63 - protein, 17 aa, Mus musculus
YINPSSGYTEYNQKFKD

SEQ ID NO: 64 - protein, 8 aa, Mus musculus
INPSSGYT

SEQ ID NO: 65 - protein, 8 aa, Mus musculus
GSSRGFDY

SEQ ID NO: 66 - protein, 6 aa, Mus musculus
SSRGFD

SEQ ID NO: 67 - protein, 10 aa, Mus musculus
VRGSSRGFDY

SEQ ID NO: 68 - protein, 11 aa, Mus musculus
RASENIYSNLA

SEQ ID NO: 69 - protein, 6 aa, Mus musculur
ENIYSN

SEQ ID NO: 70 - protein, 7 aa, mus musculur
AATNLAD

SEQ ID NO: 71 - protein, 9 aa, Mus musculus
QHFWGTPRT

SEQ ID NO: 72 - protein, 6 aa, Mus musculus
FWGTPR

SEQ ID NO: 73 - protein, 5 aa, Mus musculus
SSWMH

SEQ ID NO: 74 - protein, 7 aa, Mus musculus
GYTFTSS

SEQ ID NO: 75 - protein, 8 aa, Mus musculus
GYTFTSSW

SEQ ID NO: 76 - protein, 17 aa, Mus musculus
HIHPNSGISNYNEKFKG

SEQ ID NO: 77 - protein, 8 aa, Mus musculus
IHPNSGIS

SEQ ID NO: 78 - protein, 6 aa, Mus musculus
GGRFDD

SEQ ID NO: 79 - protein, 8 aa, Mus musculus
ARGGRFDD

SEQ ID NO: 80 - protein, 11 aa, Mus musculus
RASQSISDYLH

SEQ ID NO: 81 - protein, 11 aa, Mus musculus
GRFDSQSISDY

SEQ ID NO: 82 - protein, 10 aa, Mus musculus
QNGHSFLMYT

SEQ ID NO: 83 - protein, 7 aa, Mus musculus
GHSFLMY

SEQ ID NO: 84 - protein, 13 aa, Mus musculus
YASQNGHSFLMYT

SEQ ID NO: 85 - protein, 6 aa, mus musculus
SDYAWN

SEQ ID NO: 86 - protein, 8 aa, Mus musculus
GYSITSDY

SEQ ID NO: 87 - protein, 9 aa, Mus musculus
GYSITSDYA

SEQ ID NO: 88 - protein, 16 aa, Mus musculus
YITYSGSTNYNPSLKS

SEQ ID NO: 89 - protein, 11 aa, Mus musculus
CWDYALYAMDC

SEQ ID NO: 90 - protein, 9 aa, mus musculus
WDYALYAMD

SEQ ID NO: 91 - protein, 13 aa, Mus musculus
ARCWDYALYAMDC

SEQ ID NO: 92 - protein, 11 aa, Mus musculus
RTSENIYSYLA

SEQ ID NO: 93 - protein, 7 aa, Mus musculus
NAKTLAE

SEQ ID NO: 94 - protein, 9 aa, Mus musculus
QHHYDTPLT

SEQ ID NO: 95 - protein, 9 aa, mus musculus
NAKHYDTPL

SEQ ID NO: 96 - protein, 9 aa, Mus musculus
QHHYDTPLT

SEQ ID NO: 97 - protein, 5 aa, Mus musculus
NYGMN

SEQ ID NO: 98 - protein, 7 aa, mus musculus
GYTFTNY

SEQ ID NO: 99 - protein, 8 aa, mus musculus
GYTFTNYG

SEQ ID NO: 100 - protein, 17 aa, mus musculus
WINTNTGEPTYAEEFKG

SEQ ID NO: 101 - protein, 8 aa, Mus musculus
INTNTGEP

SEQ ID NO: 102 - protein, 8 aa, Mus musculus
DYLYYFDY

SEQ ID NO: 103 - protein, 6 aa, mus musculus
YLYYFD

SEQ ID NO: 104 - protein, 10 aa, Mus musculus
ARDYLYYFDY

SEQ ID NO: 105 - protein, 11 aa, Mus musculus
KASENVVTYVS

SEQ ID NO: 106 - protein, 7 aa, Mus musculus
SENVVTY

SEQ ID NO: 107 - protein, 6 aa, Mus musculus
ENVVTY

SEQ ID NO: 108 - protein, 7 aa, Mus musculus
GASNRYT

SEQ ID NO: 109 - protein, 9 aa, mus musculus
GQGYSYPYT

SEQ ID NO: 110 - protein, 6 aa, mus musculus
GYSYPY

SEQ ID NO: 111 - protein, 9 aa, mus musculus
GQGYSYPYT

SEQ ID NO: 112 - protein, 227 aa, homo sapiens
GQPREPQVYTLPPSREEMTKNQVSLTCLVKGFYPSDIAVEWESNGQPENNYKTTPPVLDSDGSFFLYSKLTVDKSRWQQGNVFSCSVMHEALHNHYTQKSLSLSPGGGGGSGGGGSGGGGSGQPREPQVYTLPPSREEMTKNQVSLTCLVKGFYPSDIAVEWESNGQPENNYKTTPPVLDSDGSFFLYSKLTVDKSRWQQGNVFSCSVMHEALHNHYTQKSLSLSPG

SEQ ID NO: 113 - DNA, 333 bp, mus musculus
gacattcagctgacccaatctccagcttctttggctgtgtctctagggcagagggccaccatctcctgcaaggccagccaaagtgttgattatgatggtgatagttatttgaactggtaccaacagataccaggacagccacccaaactcctcatctatgatgcatccaatctagtatctgggattccacccaggtttagtggcagtgggtctgggacagacttcaccctcaacatccatcctgtggagaaggtggatgctgcaacctatcactgtcagcaaagtactgaggacccttggacgttcggtggaggcaccaagctggaaatcaaa

SEQ ID NO: 114 - protein, 111 aa, mus musculus
DIQLTQSPASLAVSLGQRATISCKASQSVDYDGDSYLNWYQQIPGQPPKLLIYDASNLVSGIPPRFSGSGSGTDFTLNIHPVEKVDAATYHCQQSTEDPWTFGGGTKLEIK

SEQ ID NO: 115 - DNA, 372 bp, mus musculus
caggttcagctgcagcagtctggggctgagctggtgcggcctgggtcctcagtgaagatttcctgcaaagcatctggctacgcattcagtagctactggatgaactgggtgaagcagaggcctggacagggtcttgagtggattggacagatttggcctggagatggtgatactaactacaacggaaagttcaagggcaaggccacactgactgcagacgaatcctccagcacagcctacatgcagctcagcagcctggcctctgaggactctgcggtctatttctgtgcaagacgagaaacgaccactgtcgggcgttattactatgctatggactactggggtcaaggaaccacagtcaccgtctcctca

SEQ ID NO: 116 - protein, 124 aa, Mus musculus
QVQLQQSGAELVRPGSSVKISCKASGYAFSSYWMNWVKQRPGQGLEWIGQIWPGDGDTNYNGKFKGKATLTADESSSTAYMQLSSLASEDSAVYFCARRETTTVGRYYYAMDYWGQGTTVTVSS

SEQ ID NO: 117 - DNA, 648 bp, homo sapiens
gcacctgaactcctggggggaccgtcagtcttcctcttccccccaaaacccaaggacaccctcatgatctcccggacccctgaggtcacatgcgtggtggtggacgtgagccacgaagaccctgaggtcaagttcaactggtacgtggacggcgtggaggtgcataatgccaagacaaagccgcgggaggagcagtacaacagcacgtaccgtgtggtcagcgtcctcaccgtcctgcaccaggactggctgaatggcaaggagtacaagtgcaaggtctccaacaaagccctcccagcccccatcgagaaaaccatctccaaagccaaagggcagccccgagaaccacaggtgtacaccaagcccccatcccgggaggagatgaccaagaaccaggtcagcctgtcctgcctggtcaaaggcttctatcccagcgacatcgccgtggagtgggagagcaatgggcagccggagaacaactacaagaccacggttcccgtgctggactccgacggctccttccgcctcgctagctacctcaccgtggacaagagcaggtggcagcaggggaacgtcttctcatgctccgtgatgcatgaggctctgcacaaccactacacgcagaagagcctctccctgtccccgggg

SEQ ID NO: 118 - protein, 718 aa, Artificial
  Chimeric homo sapiens mus musculus
DIQLTQSPASLAVSLGQRATISCKASQSVDYDGDSYLNWYQQIPGQPPKLLIYDASNLVSGIPPRFSGSGSGTDFTLNIHPVEKVDAATYHCQQSTEDPWTFGGGTKLEIKGGGGSGGGGSGGGGSQVQLQQSGAELVRPGSSVKISCKASGYAFSSYWMNWVKQRPGQGLEWIGQIWPGDGDTNYNGKFKGKATLTADESSSTAYMQLSSLASEDSAVYFCARRETTTVGRYYYAMDYWGQGTTVTVSSGGGSSAPELLGGPSVFLFPPKPKDTLMISRTPEVTCVVVDVSHEDPEVKFNWYVDGVEVHNAKTKPREEQYNSTYRVVSVLTVLHQDWLNGKEYKCKVSNKALPAPIEKTISKAKGQPREPQVYTKPPSREEMTKNQVSLSCLVKGFYPSDIAVEWESNGQPENNYKTTVPVLDSDGSFRLASYLTVDKSRWQQGNVFSCSVMHEALHNHYTQKSLSLSPGSTGSDIKLQQSGAELARPGASVKMSCKTSGYTFTRYTMHWVKQRPGQGLEWIGYINPSRGYTNYNQKFKDKATLTTDKSSSTAYMQLSSLTSEDSAVYYCARYYDDHYCLDYWGQGTTLTVSSVEGGSGGSGGSGGSGGVDDIQLTQSPAIMSASPGEKVTMTCRASSSVSYMNWYQQKSGTSPKRWIYDTSKVASGVPYRFSGSGSGTSYSLTISSMEAEDAATYYCQQWSSNPLTFGAGTKLELK

SEQ ID NO: 119 - protein, 249 aa, mus musculus
STGSQVQLQQSGPELVKPGASVKMSCKASGYTFTDYVINWGKQRSGQGLEWIGEIYPGSGTNYYNEKFKAKATLTADKSSNIAYMQLSSLTSEDSAVYFCARRGRYGLYAMDYWGQGTSVTVSSVEGGSGGSGGSGGSGGVDDIQMTQTTSSLSASLGDRVTISCRASQDISNYLNWYQQKPDGTVKLLIYYTSRLHSGVPSRFSGSGSGTDYSLTINNLEQEDIATYFCQQGNTRPWTFGGGTKLEIK

SEQ ID NO: 120 - protein, 251 aa, mus musculus
STGSEVQLQESGPGLVKPSQSLSLTCTVTGYSITSDYAWNWIRQFPGNKLEWMGYITYSGSTSYNPSLESRISITRDTSTNQFFLQLNSVTTEDTATYYCARGGYYGSSWGVFAYWGQGTLVTVSAVEGGSGGSGGSGGSGGVDDIQMTQSPASLSASVGETVTITCRVSENIYSYLAWYQQKQGKSPQLLVYNAKTLAEGVPSRFSGSGSGTQFSLKINSLQPEDFGSYYCQHHYGTPWTFGGGTKLEIK

SEQ ID NO: 121 - protein, 245 aa, mus musculus
STGSEVQLQQSGPELVKPGASVKISCKTSGYTFTEYTMHWVKQSHGKSLEWIGGISPNIGGTSYNQKFKGKATLTVDKSSSTAYMELRSLTSEDSAVYYCARRGGSFDYWGQGTTLTVSSVEGGSGGSGGSGGSGGVDDIVMTQSPATLSVTPGDRVSLSCRASQSISDYLHWYQQKSHESPRLLIKYASQSISGIPSRFSGSGSGSDFTLSINSVEPEDVGVYYCQNGHSFPLTFGAGTKLELK

SEQ ID NO: 122 - protein, 246 aa, Mus musculus
STGSQVQLQQSAVELARPGASVKMSCKASGYTFTSFTMHWVKQRPGQGLEWIGYINPSSGYTEYNQKFKDKTTLTADKSSSTAYMQLDSLTSDDSAVYYCVRGSSRGFDYWGQGTLVTVSAVEGGSGGSGGSGGSGGVDDIQMIQSPASLSVSVGETVTITCRASENIYSNLAWFQQKQGKSPQLLVYAATNLADGVPSRFSGSGSGTQYSLKINSLQSEDFGIYYCQHFWGTPRTFGGGTKLEIK

SEQ ID NO: 123 - protein, 245 aa, Mus musculus
STGSQVQLQQPGSVLVRPGASVKLSCKASGYTFTSSWMHWAKQRPGQGLEWIGHIHPNSGISNYNEKFKGKATLTVDTSSSTAYVDLSSLTSEDSAVYYCARGGRFDDWGAGTTVTVSSVEGGSGGSGGSGGSGGVDDIVMTQSPATLSVTPGDRVSLSCRASQSISDYLHWYQQKSHESPRLLIKYASQSISGIPSRFSGSGSGSDFTLSINSVEPEDVGVYYCQNGHSFLMYTFGGGTKLEIK

SEQ ID NO: 124 - protein, 249 aa, Mus musculus
STGSDVQLQESGPGLVKPSQSLSLTCTVTGYSITSDYAWNWIRQFPGNKLEWMGYITYSGSTNYNPSLKSRISITRDTSKNQFFLQLNSVTTEDTATYYCARCWDYALYAMDCWGQGTSVTVSSVEGGSGGSGGSGGSGGVDDIQMTQSPASLSASVGETVTITCRTSENIYSYLAWCQQKQGKSPQLLVYNAKTLAEGVPSRFSGSGSGTHFSLKINSLQPEDFGIYYCQHHYDTPLTFGAGTKLELK

SEQ ID NO: 125 - protein, 246 aa, Mus musculus
STGSQIQLVQSGPELQKPGETVKISCKASGYTFTNYGMNWVKQAPGKGLKWMGWINTNTGEPTYAEEFKGRFAFSLETSASTAYLQINNLKNEDTATYFCARDYLYYFDYWGQGTTLTVSSVEGGSGGSGGSGGSGGVDNIVMTQSPKSMSMSVGERVTLTCKASENVVTYVSWYQQKPEQSPKLLIYGASNRYTGVPDRFTGSGSATDFTLTISSVQAEDLADYHCGQGYSYPYTFGGGTKLEIK

SEQ ID NO: 126 - DNA, 751 bp, mus musculus
gtcgactggaagccaggtacagctgcagcagtctggccctgaactcgtcaaaccaggagcttccgtgaagatgtcctgcaaggcttcagggtacacgtttaccgactatgtgatcaattggggtaagcagcgctctgggcaaggcttggagtggattggcgagatctatcctgggagtgggaccaactattacaacgagaagttcaaggccaaagccactttgactgcagacaagagctcaaacattgcctacatgcaactgagctccctgacatcagaggattctgctgtgtacttctgtgcacgtagaggtcggtacggtctgtatgccatggactattggggccaaggcacttccgtgacagtcagctctgtggaaggaggaagtggcggttcaggaggtagcggagggtccggaggagtggatgacattcagatgacacagaccacttctagcctctccgcatcccttggggatagggtcaccatcagttgtagggctagccaggacatttccaattacctgaactggtatcagcagaaacccgatggcacagttaagcttctgatctactacacaagcagactgcactcaggggttccatctcggtttagtggaagtggctctggtaccgactattccctgaccatcaacaatctggaacaggaagatatcgccacctacttctgccaacagggcaatactcgaccctggacatttggtggcggcacgaaactcgagataaaataa

SEQ ID NO: 127 - DNA, 757 bp, Mus musculus
gtcgactggatccgaggtacagttgcaggagagtgggcctggactggtcaaaccctcccaatctctgagcttgacatgcacagtcacaggctacagcatcacctccgactacgcttggaattggattcgacagtttcccggcaacaagctggaatggatgggctacatcacctatagtggtagcacttcctataatccctcacttgagagccggatttccatcactagggatacgagcaccaaccagttcttcctgcagctgaatagcgtcaccaccgaagatactgccacctattactgcgcaagaggcggttactatggcagttcatggggtgtattcgcctattggggacaggggacacttgtgacagtgtctgctgttgaaggtggatccggcggatcaggagggagtggtggcagtggaggtgttgacgacattcagatgacccaatcccctgcttctctctcagcctctgtgggagagactgtgaccataacctgtcgtgttagcgagaacatctactcctatctcgcctggtatcagcagaaacaggggaaatccccacaactgctcgtgtacaatgccaagactctggcagaaggagtgccaagccgcttttccgggtctgggtctgggacacagttctcactgaagatcaactctttgcaacctgaggattttggctcttactactgtcagcatcactatggcacaccatggacgtttggtggcggcactaagctggagattaagtaa

SEQ ID NO: 128 - DNA, 739 bp, Mus musculus
gtcgactgggtccgaagtgcaactgcaacagtctggccctgagctggtcaaacccggtgcttcagtgaagatctcctgcaagacatccggctacaccttcactgagtacaccatgcactgggtcaaacagtctcacggtaagagcctggagtggataggcggaatttcacccaacattggagggacctcctataaccagaagttcaagggcaaagccacccttacagttgacaagagcagttcaactgcctacatggaactgcgctcattgacctccgaggattcagccgtgtattactgcgctagaaggggaggatccttcgattattggggccaaggcactacgcttaccgtgagcagcgttgaaggtggttctggcggctctggtggaagtggagggagtggcggggtagacgacatcgtgatgactcagagtccagcaactctgtccgttacacctggagatcgagtgtctctgagttgtcgtgcaagccagtctatctctgactatctgcactggtatcagcagaagagccatgagtcacctaggctgttgatcaagtacgcctctcagtccattagcgggattccatcccggtttagtggctctggctccggtagtgacttcacactcagcatcaatagcgtcgaaccagaggatgtaggggtgtactactgtcagaatgggcattcctttcccctcacatttggagctggtaccaaactcgagctgaaataa

SEQ ID NO: 129 - DNA, 742 bp, Mus musculus
gtcgactggctcccaagtacagcttcagcagtctgccgtcgaacttgctcgaccaggagcttcagtgaagatgagctgcaaagcctctggttacaccttcacgtcctttaccatgcattgggtgaagcagcgtcctggccaaggcctggagtggattggctacatcaatccctccagcgggtataccgagtacaaccagaagttcaaggacaaaacaaccctgactgccgataagtcaagtagcacagcctatatgcagctggattccctgacatcagacgatagcgctgtgtattactgcgttaggggctctagcagagggttcgactattggggtcaaggcacactggtcacggttagtgccgttgaaggaggctctggaggcagtggaggttctggagggtcaggcggtgtggatgacattcagatgattcagagtcccgctagcttgagtgtaagcgtcggtgagacagtgaccatcacttgtcgcgcatccgaaaacatctactccaatctcgcatggttccagcagaaacagggcaaatcaccccaattgctcgtgtatgccgcaactaatctggctgatggtgtgccttccaggtttagcgggtctggatctgggactcagtactccctgaagatcaactccctccagtctgaggacttcgggatctattactgtcagcacttttggggaactccacggacctttggaggcgggaccaaactggagataaagtaa

SEQ ID NO: 130 - DNA, 696 bp, Mus musculus
ctggtgaggccaggtgcatctgtgaagctgtcatgcaaagcatccgggtacacgttcacctcttcatggatgcattgggccaaacagcgtccaggccagggccttgagtggattggacacattcaccccaatagcggcatatccaactacaacgagaagttcaagggcaaagccacactgacagtggatacttccagctctacagcctatgtggaccttagtagcttgaccagtgaggattctgccgtatactactgtgctagaggtgggcggtttgacgattggggtgctgggaccacagtcaccgtgagcagtgtcgaaggtggatcaggtggatctggaggctcaggcggttctggcggtgttgacgacatcgtgatgactcaaagccctgctactctctctgtcacacccggagatagggtaagcctcagttgtcgagcaagccagtcaatcagcgactatctgcactggtatcagcagaagtcccatgaatccccacgcttgctcatcaagtacgccagtcagtccatcagtggcattccttcccggttttctgggtctggatccgggtcagacttcactctgagcattaactccgtcgaacccgaggatgttggcgtgtattattgccagaatggacattccttcctgatgtacacctttggcggagggaccaaactggagatcaagtaa

SEQ ID NO: 131 - DNA, 751 bp, Mus musculus
gtcgactgggtctgatgtgcagttgcaggagtcaggacctgggcttgtcaagccaagccagagcctcagtctcacttgcactgtcacaggctatagcatcacatccgactatgcttggaattggattaggcagtttcctggcaataagctggaatggatggggtacatcacctattccggcagtaccaactacaatcccagcttgaaatctcggatttccataacacgcgatactagcaagaaccagttcttccttcagctgaactctgtgacaacagaggataccgctacgtactattgcgccagatgctgggattacgccctgtatgccatggactgttggggtcaaggtaccagcgttactgtgtctagcgtcgaaggcggaagtggcggctcaggagggtcaggaggctcaggcggagtggatgacattcagatgacccaatctcccgcatccctgtccgcatcagtaggggagacagtgaccattacctgtcgtacttccgagaacatctactcctatcttgcctggtgtcaacagaaacaggggaaaagtccacagctgctggtgtataacgccaagaccttggcagaaggtgttcccagtcgattctctggttccggatccggtacacacttcagcctgaagatcaattctctgcaaccagaggactttggaatctactactgccagcatcactacgacactcctctgacgtttggcgctggtaccaagctcgaactgaaataa

SEQ ID NO: 132 - DNA, 742 bp, Mus musculus
gtcgactggtagccagatacagctggtacagtcaggaccagagctgcagaaacctggagagacagtgaagatcagctgcaaggctagcgggtacaccttcacgaattacgggatgaactgggtcaagcaggctccaggcaaagggctgaagtggatgggctggattaacaccaatactggggaaccaacctatgccgaggaattcaaggggagatttgccttttccctcgaaaccagcgcctcaaccgcctatctccagatcaacaacctgaagaatgaggataccgctacctacttctgtgcaagggactacctctactacttcgactattggggccaaggtacgactcttacagtctctagtgttgagggagggagtggaggttctggaggctctggtggctctggaggcgttgacaacatcgtgatgactcagtctcccaaaagcatgagtatgagtgtgggtgaacgagttaccttgacatgcaaagcctccgagaatgtcgtgacatacgtgtcctggtatcagcagaaacccgagcaatcccctaagctgctgatctatggcgctagcaatcgctatactggcgtacctgatcggttcacaggatcaggctcagccactgactttactcttaccatttcctccgtgcaggcagaagatttggcagattaccactgtgggcaaggttactcttatccctatacatttggaggcggcacaaagctggagattaagtaa

SEQ ID NO: 133 - protein, 720 aa, Artificial
  Chimeric homo sapiens mus musculus
DIQLTQSPASLAVSLGQRATISCKASQSVDYDGDSYLNWYQQIPGQPPKLLIYDASNLVSGIPPRFSGSGSGTDFTLNIHPVEKVDAATYHCQQSTEDPWTFGGGTKLEIKGGGGSGGGGSGGGGSQVQLQQSGAELVRPGSSVKISCKASGYAFSSYWMNWVKQRPGQGLEWIGQIWPGDGDTNYNGKFKGKATLTADESSSTAYMQLSSLASEDSAVYFCARRETTTVGRYYYAMDYWGQGTTVTVSSGGGSSAPELLGGPSVFLFPPKPKDTLMISRTPEVTCVVVDVSHEDPEVKFNWYVDGVEVHNAKTKPREEQYNSTYRVVSVLTVLHQDWLNGKEYKCKVSNKALPAPIEKTISKAKGQPREPQVYTKPPSREEMTKNQVSLSCLVKGFYPSDIAVEWESNGQPENNYKTTVPVLDSDGSFRLASYLTVDKSRWQQGNVFSCSVMHEALHNHYTQKSLSLSPGSTGSQVQLQQSGPELVKPGASVKMSCKASGYTFTDYVINWGKQRSGQGLEWIGEIYPGSGTNYYNEKFKAKATLTADKSSNIAYMQLSSLTSEDSAVYFCARRGRYGLYAMDYWGQGTSVTVSSVEGGSGGSGGSGGSGGVDDIQMTQTTSSLSASLGDRVTISCRASQDISNYLNWYQQKPDGTVKLLIYYTSRLHSGVPSRFSGSGSGTDYSLTINNLEQEDIATYFCQQGNTRPWTFGGGTKLEIK

SEQ ID NO: 134 - protein, 722 aa, Artificial
  Chimeric homo sapiens mus musculus
DIQLTQSPASLAVSLGQRATISCKASQSVDYDGDSYLNWYQQIPGQPPKLLIYDASNLVSGIPPRFSGSGSGTDFTLNIHPVEKVDAATYHCQQSTEDPWTFGGGTKLEIKGGGGSGGGGSGGGGSQVQLQQSGAELVRPGSSVKISCKASGYAFSSYWMNWVKQRPGQGLEWIGQIWPGDGDTNYNGKFKGKATLTADESSSTAYMQLSSLASEDSAVYFCARRETTTVGRYYYAMDYWGQGTTVTVSSGGGSSAPELLGGPSVFLFPPKPKDTLMISRTPEVTCVVVDVSHEDPEVKFNWYVDGVEVHNAKTKPREEQYNSTYRVVSVLTVLHQDWLNGKEYKCKVSNKALPAPIEKTISKAKGQPREPQVYTKPPSREEMTKNQVSLSCLVKGFYPSDIAVEWESNGQPENNYKTTVPVLDSDGSFRLASYLTVDKSRWQQGNVFSCSVMHEALHNHYTQKSLSLSPGSTGSEVQLQESGPGLVKPSQSLSLTCTVTGYSITSDYAWNWIRQFPGNKLEWMGYITYSGSTSYNPSLESRISITRDTSTNQFFLQLNSVTTEDTATYYCARGGYYGSSWGVFAYWGQGTLVTVSAVEGGSGGSGGSGGSGGVDDIQMTQSPASLSASVGETVTITCRVSENIYSYLAWYQQKQGKSPQLLVYNAKTLAEGVPSRFSGSGSGTQFSLKINSLQPEDFGSYYCQHHYGTPWTFGGGTKLEIK

SEQ ID NO: 135 - protein, 716 aa, Artificial
  Chimeric homo sapiens mus musculus
DIQLTQSPASLAVSLGQRATISCKASQSVDYDGDSYLNWYQQIPGQPPKLLIYDASNLVSGIPPRFSGSGSGTDFTLNIHPVEKVDAATYHCQQSTEDPWTFGGGTKLEIKGGGGSGGGGSGGGGSQVQLQQSGAELVRPGSSVKISCKASGYAFSSYWMNWVKQRPGQGLEWIGQIWPGDGDTNYNGKFKGKATLTADESSSTAYMQLSSLASEDSAVYFCARRETTTVGRYYYAMDYWGQGTTVTVSSGGGSSAPELLGGPSVFLFPPKPKDTLMISRTPEVTCVVVDVSHEDPEVKFNWYVDGVEVHNAKTKPREEQYNSTYRVVSVLTVLHQDWLNGKEYKCKVSNKALPAPIEKTISKAKGQPREPQVYTKPPSREEMTKNQVSLSCLVKGFYPSDIAVEWESNGQPENNYKTTVPVLDSDGSFRLASYLTVDKSRWQQGNVFSCSVMHEALHNHYTQKSLSLSPGSTGSEVQLQQSGPELVKPGASVKISCKTSGYTFTEYTMHWVKQSHGKSLEWIGGISPNIGGTSYNQKFKGKATLTVDKSSSTAYMELRSLTSEDSAVYYCARRGGSFDYWGQGTTLTVSSVEGGSGGSGGSGGSGGVDDIVMTQSPATLSVTPGDRVSLSCRASQSISDYLHWYQQKSHESPRLLIKYASQSISGIPSRFSGSGSGSDFTLSINSVEPEDVGVYYCQNGHSFPLTFGAGTKLELK

SEQ ID NO: 136 - protein, 717 aa, Artificial
  Chimeric homo sapiens mus musculus
DIQLTQSPASLAVSLGQRATISCKASQSVDYDGDSYLNWYQQIPGQPPKLLIYDASNLVSGIPPRFSGSGSGTDFTLNIHPVEKVDAATYHCQQSTEDPWTFGGGTKLEIKGGGGSGGGGSGGGGSQVQLQQSGAELVRPGSSVKISCKASGYAFSSYWMNWVKQRPGQGLEWIGQIWPGDGDTNYNGKFKGKATLTADESSSTAYMQLSSLASEDSAVYFCARRETTTVGRYYYAMDYWGQGTTVTVSSGGGSSAPELLGGPSVFLFPPKPKDTLMISRTPEVTCVVVDVSHEDPEVKFNWYVDGVEVHNAKTKPREEQYNSTYRVVSVLTVLHQDWLNGKEYKCKVSNKALPAPIEKTISKAKGQPREPQVYTKPPSREEMTKNQVSLSCLVKGFYPSDIAVEWESNGQPENNYKTTVPVLDSDGSFRLASYLTVDKSRWQQGNVFSCSVMHEALHNHYTQKSLSLSPGSTGSQVQLQQSAVELARPGASVKMSCKASGYTFTSFTMHWVKQRPGQGLEWIGYINPSSGYTEYNQKFKDKTTLTADKSSSTAYMQLDSLTSDDSAVYYCVRGSSRGFDYWGQGTLVTVSAVEGGSGGSGGSGGSGGVDDIQMIQSPASLSVSVGETVTITCRASENIYSNLAWFQQKQGKSPQLLVYAATNLADGVPSRFSGSGSGTQYSLKINSLQSEDFGIYYCQHFWGTPRTFGGGTKLEIK

SEQ ID NO: 137 - protein, 716 aa, Artificial
  Chimeric homo sapiens mus musculus
DIQLTQSPASLAVSLGQRATISCKASQSVDYDGDSYLNWYQQIPGQPPKLLIYDASNLVSGIPPRFSGSGSGTDFTLNIHPVEKVDAATYHCQQSTEDPWTFGGGTKLEIKGGGGSGGGGSGGGGSQVQLQQSGAELVRPGSSVKISCKASGYAFSSYWMNWVKQRPGQGLEWIGQIWPGDGDTNYNGKFKGKATLTADESSSTAYMQLSSLASEDSAVYFCARRETTTVGRYYYAMDYWGQGTTVTVSSGGGSSAPELLGGPSVFLFPPKPKDTLMISRTPEVTCVVVDVSHEDPEVKFNWYVDGVEVHNAKTKPREEQYNSTYRVVSVLTVLHQDWLNGKEYKCKVSNKALPAPIEKTISKAKGQPREPQVYTKPPSREEMTKNQVSLSCLVKGFYPSDIAVEWESNGQPENNYKTTVPVLDSDGSFRLASYLTVDKSRWQQGNVFSCSVMHEALHNHYTQKSLSLSPGSTGSQVQLQQPGSVLVRPGASVKLSCKASGYTFTSSWMHWAKQRPGQGLEWIGHIHPNSGISNYNEKFKGKATLTVDTSSSTAYVDLSSLTSEDSAVYYCARGGRFDDWGAGTTVTVSSVEGGSGGSGGSGGSGGVDDIVMTQSPATLSVTPGDRVSLSCRASQSISDYLHWYQQKSHESPRLLIKYASQSISGIPSRFSGSGSGSDFTLSINSVEPEDVGVYYCQNGHSFLMYTFGGGTKLEIK

SEQ ID NO: 138 - protein, 720 aa, Artificial
  Chimeric homo sapiens mus musculus
DIQLTQSPASLAVSLGQRATISCKASQSVDYDGDSYLNWYQQIPGQPPKLLIYDASNLVSGIPPRFSGSGSGTDFTLNIHPVEKVDAATYHCQQSTEDPWTFGGGTKLEIKGGGGSGGGGSGGGGSQVQLQQSGAELVRPGSSVKISCKASGYAFSSYWMNWVKQRPGQGLEWIGQIWPGDGDTNYNGKFKGKATLTADESSSTAYMQLSSLASEDSAVYFCARRETTTVGRYYYAMDYWGQGTTVTVSSGGGSSAPELLGGPSVFLFPPKPKDTLMISRTPEVTCVVVDVSHEDPEVKFNWYVDGVEVHNAKTKPREEQYNSTYRVVSVLTVLHQDWLNGKEYKCKVSNKALPAPIEKTISKAKGQPREPQVYTKPPSREEMTKNQVSLSCLVKGFYPSDIAVEWESNGQPENNYKTTVPVLDSDGSFRLASYLTVDKSRWQQGNVFSCSVMHEALHNHYTQKSLSLSPGSTGSDVQLQESGPGLVKPSQSLSLTCTVTGYSITSDYAWNWIRQFPGNKLEWMGYITYSGSTNYNPSLKSRISITRDTSKNQFFLQLNSVTTEDTATYYCARCWDYALYAMDCWGQGTSVTVSSVEGGSGGSGGSGGSGGVDDIQMTQSPASLSASVGETVTITCRTSENIYSYLAWCQQKQGKSPQLLVYNAKTLAEGVPSRFSGSGSGTHFSLKINSLQPEDFGIYYCQHHYDTPLTFGAGTKLELK

SEQ ID NO: 139 - protein, 717 aa, Artificial
  Chimeric homo sapiens mus musculus
DIQLTQSPASLAVSLGQRATISCKASQSVDYDGDSYLNWYQQIPGQPPKLLIYDASNLVSGIPPRFSGSGSGTDFTLNIHPVEKVDAATYHCQQSTEDPWTFGGGTKLEIKGGGGSGGGGSGGGGSQVQLQQSGAELVRPGSSVKISCKASGYAFSSYWMNWVKQRPGQGLEWIGQIWPGDGDTNYNGKFKGKATLTADESSSTAYMQLSSLASEDSAVYFCARRETTTVGRYYYAMDYWGQGTTVTVSSGGGSSAPELLGGPSVFLFPPKPKDTLMISRTPEVTCVVVDVSHEDPEVKFNWYVDGVEVHNAKTKPREEQYNSTYRVVSVLTVLHQDWLNGKEYKCKVSNKALPAPIEKTISKAKGQPREPQVYTKPPSREEMTKNQVSLSCLVKGFYPSDIAVEWESNGQPENNYKTTVPVLDSDGSFRLASYLTVDKSRWQQGNVFSCSVMHEALHNHYTQKSLSLSPGSTGSQIQLVQSGPELQKPGETVKISCKASGYTFTNYGMNWVKQAPGKGLKWMGWINTNTGEPTYAEEFKGRFAFSLETSASTAYLQINNLKNEDTATYFCARDYLYYFDYWGQGTTLTVSSVEGGSGGSGGSGGSGGVDNIVMTQSPKSMSMSVGERVTLTCKASENVVTYVSWYQQKPEQSPKLLIYGASNRYTGVPDRFTGSGSATDFTLTISSVQAEDLADYHCGQGYSYPYTFGGGTKLEIK

SEQ ID NO: 140 - protein, 698 aa, Artificial
  Chimeric homo sapiens mus musculus
DIQLTQSPASLAVSLGQRATISCKASQSVDYDGDSYLNWYQQIPGQPPKLLIYDASNLVSGIPPRFSGSGSGTDFTLNIHPVEKVDAATYHCQQSTEDPWTFGGGTKLEIKGGGGSGGGGSGGGGSQVQLQQSGAELVRPGSSVKISCKASGYAFSSYWMNWVKQRPGQGLEWIGQIWPGDGDTNYNGKFKGKATLTADESSSTAYMQLSSLASEDSAVYFCARRETTTVGRYYYAMDYWGQGTTVTVSSGGGSSAPELLGGPSVFLFPPKPKDTLMISRTPEVTCVVVDVSHEDPEVKFNWYVDGVEVHNAKTKPREEQYNSTYRVVSVLTVLHQDWLNGKEYKCKVSNKALPAPIEKTISKAKGQPREPQVYTKPPSREEMTKNQVSLSCLVKGFYPSDIAVEWESNGQPENNYKTTVPVLDSDGSFRLASYLTVDKSRWQQGNVFSCSVMHEALHNHYTQKSLSLSPGSTGSEVQLQQSGPELVKPGASVKISCKTSGYTFTEYTMHWVKQSHGKSLEWIGGISPNIGGTSYNQKFKGKATLTVDKSSSTAYMELRSLTSEDSAVYYCARRGGSFDYWGQGTTLTVSSASTKGPSVFPLAPSSKSTSGGTAALGCLVKDYFPEPVTVSWNSGALTSGVHTFPAVLQSSGLYSLSSVVTVPSSSLGTQTYICNVNHKPSNTKVDKRVEPKSCDKTH

SEQ ID NO: 141 - protein, 214 aa, Artificial
  Chimeric homo sapiens mus musculus
DIVMTQSPATLSVTPGDRVSLSCRASQSISDYLHWYQQKSHESPRLLIKYASQSISGIPSRFSGSGSGSDFTLSINSVEPEDVGVYYCQNGHSFPLTFGAGTKLELKRTVAAPSVFIFPPSDEQLKSGTASVVCLLNNFYPREAKVQWKVDNALQSGNSQESVTEQDSKDSTYSLSSTLTLSKADYEKHKVYACEVTHQGLSSPVTKSFNRGEC

SEQ ID NO: 142 - protein, 837 aa, Artificial
  Chimeric homo sapiens mus musculus
DIQLTQSPASLAVSLGQRATISCKASQSVDYDGDSYLNWYQQIPGQPPKLLIYDASNLVSGIPPRFSGSGSGTDFTLNIHPVEKVDAATYHCQQSTEDPWTFGGGTKLEIKGGGGSGGGGSGGGGSQVQLQQSGAELVRPGSSVKISCKASGYAFSSYWMNWVKQRPGQGLEWIGQIWPGDGDTNYNGKFKGKATLTADESSSTAYMQLSSLASEDSAVYFCARRETTTVGRYYYAMDYWGQGTTVTVSSGGGSSAPELLGGPSVFLFPPKPKDTLMISRTPEVTCVVVDVSHEDPEVKFNWYVDGVEVHNAKTKPREEQYNSTYRVVSVLTVLHQDWLNGKEYKCKVSNKALPAPIEKTISKAKGQPREPQVYTLPPSREEMTKNQVSLTCLVKGFYPSDIAVEWESNGQPENNYKTTPPVLDSDGSFFLYSKLTVDKSRWQQGNVFSCSVMHEALHNHYTQKSLSLSPGGGGGSGGGGSGGGGSGQPREPQVYTLPPSREEMTKNQVSLTCLVKGFYPSDIAVEWESNGQPENNYKTTPPVLDSDGSFFLYSKLTVDKSRWQQGNVFSCSVMHEALHNHYTQKSLSLSPGSTGSEVQLQQSGPELVKPGASVKISCKTSGYTFTEYTMHWVKQSHGKSLEWIGGISPNIGGTSYNQKFKGKATLTVDKSSSTAYMELRSLTSEDSAVYYCARRGGSFDYWGQGTTLTVSSVEGGSGGSGGSGGSGGVDDIVMTQSPATLSVTPGDRVSLSCRASQSISDYLHWYQQKSHESPRLLIKYASQSISGIPSRFSGSGSGSDFTLSINSVEPEDVGVYYCQNGHSFPLTFGAGTKLELK

SEQ ID NO: 143 - protein, 837 aa, Artificial
  Chimeric homo sapiens mus musculus
DIQLTQSPASLAVSLGQRATISCKASQSVDYDGDSYLNWYQQIPGQPPKLLIYDASNLVSGIPPRFSGSGSGTDFTLNIHPVEKVDAATYHCQQSTEDPWTFGGGTKLEIKGGGGSGGGGSGGGGSQVQLQQSGAELVRPGSSVKISCKASGYAFSSYWMNWVKQRPGQGLEWIGQIWPGDGDTNYNGKFKGKATLTADESSSTAYMQLSSLASEDSAVYFCARRETTTVGRYYYAMDYWGQGTTVTVSSGGGSSAPELLGGPSVFLFPPKPKDTLMISRTPEVTCVVVDVSHEDPEVKFNWYVDGVEVHNAKTKPREEQYSSTYRVVSVLTVLHQDWLNGKEYKCKVSNKALPAPIEKTISKAKGQPREPQVYTLPPSREEMTKNQVSLTCLVKGFYPSDIAVEWESNGQPENNYKTTPPVLDSDGSFFLYSKLTVDKSRWQQGNVFSCSVMHEALHNHYTQKSLSLSPGGGGGSGGGGSGGGGSGQPREPQVYTLPPSREEMTKNQVSLTCLVKGFYPSDIAVEWESNGQPENNYKTTPPVLDSDGSFFLYSKLTVDKSRWQQGNVFSCSVMHEALHNHYTQKSLSLSPGSTGSEVQLQQSGPELVKPGASVKISCKTSGYTFTEYTMHWVKQSHGKSLEWIGGISPNIGGTSYNQKFKGKATLTVDKSSSTAYMELRSLTSEDSAVYYCARRGGSFDYWGQGTTLTVSSVEGGSGGSGGSGGSGGVDDIVMTQSPATLSVTPGDRVSLSCRASQSISDYLHWYQQKSHESPRLLIKYASQSISGIPSRFSGSGSGSDFTLSINSVEPEDVGVYYCQNGHSFPLTFGAGTKLELK

SEQ ID NO: 144 - protein, 218 aa, Artificial
  Chimeric homo sapiens mus musculus
DIQLTQSPASLAVSLGQRATISCKASQSVDYDGDSYLNWYQQIPGQPPKLLIYDASNLVSGIPPRFSGSGSGTDFTLNIHPVEKVDAATYHCQQSTEDPWTFGGGTKLEIKRTVAAPSVFIFPPSDEQLKSGTASVVCLLNNFYPREAKVQWKVDNALQSGNSQESVTEQDSKDSTYSLSSTLTLSKADYEKHKVYACEVTHQGLSSPVTKSFNRGEC

SEQ ID NO: 145 - protein, 675 aa, Artificial
  Chimeric homo sapiens mus musculus
QVQLQQSGAELVRPGSSVKISCKASGYAFSSYWMNWVKQRPGQGLEWIGQIWPGDGDTNYNGKFKGKATLTADESSSTAYMQLSSLASEDSAVYFCARRETTTVGRYYYAMDYWGQGTTVTVSSASTKGPSVFPLAPSSKSTSGGTAALGCLVKDYFPEPVTVSWNSGALTSGVHTFPAVLQSSGLYSLSSVVTVPSSSLGTQTYICNVNHKPSNTKVDKRVEPKSCGGGSSAPELLGGPSVFLFPPKPKDTLMISRTPEVTCVVVDVSHEDPEVKFNWYVDGVEVHNAKTKPREEQYSSTYRVVSVLTVLHQDWLNGKEYKCKVSNKALPAPIEKTISKAKGQPREPQVYTKPPSREEMTKNQVSLSCLVKGFYPSDIAVEWESNGQPENNYKTTVPVLDSDGSFRLASYLTVDKSRWQQGNVFSCSVMHEALHNHYTQKSLSLSPGSTGSEVQLQQSGPELVKPGASVKISCKTSGYTFTEYTMHWVKQSHGKSLEWIGGISPNIGGTSYNQKFKGKATLTVDKSSSTAYMELRSLTSEDSAVYYCARRGGSFDYWGQGTTLTVSSRTVAAPSVFIFPPSDEQLKSGTASVVCLLNNFYPREAKVQWKVDNALQSGNSQESVTEQDSKDSTYSLSSTLTLSKADYEKHKVYACEVTHQGLSSPVTKSFNRGEC

SEQ ID NO: 146 - protein, 214 aa, Artificial
  Chimeric homo sapiens mus musculus
DIVMTQSPATLSVTPGDRVSLSCRASQSISDYLHWYQQKSHESPRLLIKYASQSISGIPSRFSGSGSGSDFTLSINSVEPEDVGVYYCQNGHSFPLTFGAGTKLELKASTKGPSVFPLAPSSKSTSGGTAALGCLVKDYFPEPVTVSWNSGALTSGVHTFPAVLQSSGLYSLSSVVTVPSSSLGTQTYICNVNHKPSNTKVDKRVEPKSCDKTH

SEQ ID NO: 147 - protein, 218 aa, Artificial; identical to SEQ ID NO: 144
  Chimeric homo sapiens mus musculus

SEQ ID NO: 148 - protein, 801 aa, Artificial
  Chimeric homo sapiens mus musculus
QVQLQQSGAELVRPGSSVKISCKASGYAFSSYWMNWVKQRPGQGLEWIGQIWPGDGDTNYNGKFKGKATLTADESSSTAYMQLSSLASEDSAVYFCARRETTTVGRYYYAMDYWGQGTTVTVSSASTKGPSVFPLAPSSKSTSGGTAALGCLVKDYFPEPVTVSWNSGALTSGVHTFPAVLQSSGLYSLSSVVTVPSSSLGTQTYICNVNHKPSNTKVDKRVEPKSCDKTHTCPPCPAPELLGGPSVFLFPPKPKDTLMISRTPEVTCVVVDVSHEDPEVKFNWYVDGVEVHNAKTKPREEQYSSTYRVVSVLTVLHQDWLNGKEYKCKVSNKALPAPIEKTISKAKGQPREPQVYTLPPSREEMTKNQVSLTCLVKGFYPSDIAVEWESNGQPENNYKTTPPVLDSDGSFFLYSKLTVDKSRWQQGNVFSCSVMHEALHNHYTQKSLSLSPGGGGGSGGGGSGGGGSGQPREPQVYTLPPSREEMTKNQVSLTCLVKGFYPSDIAVEWESNGQPENNYKTTPPVLDSDGSFFLYSKLTVDKSRWQQGNVFSCSVMHEALHNHYTQKSLSLSPGSTGSEVQLQQSGPELVKPGASVKISCKTSGYTFTEYTMHWVKQSHGKSLEWIGGISPNIGGTSYNQKFKGKATLTVDKSSSTAYMELRSLTSEDSAVYYCARRGGSFDYWGQGTTLTVSSRTVAAPSVFIFPPSDEQLKSGTASVVCLLNNFYPREAKVQWKVDNALQSGNSQESVTEQDSKDSTYSLSSTLTLSKADYEKHKVYACEVTHQGLSSPVTKSFNRGEC

SEQ ID NO: 149 - protein, 214 aa, Artificial; identical to SEQ ID NO: 146
  Chimeric homo sapiens mus musculus

SEQ ID NO: 150 - protein, 218 aa, Artificial; identical to SEQ ID NO: 144
  Chimeric homo sapiens mus musculus

SEQ ID NO: 151 - protein, 801 aa, Artificial; identical to SEQ ID NO: 148
  Chimeric homo sapiens mus musculus

SEQ ID NO: 152 - protein, 214 aa, Artificial; identical to SEQ ID NO: 146
  Chimeric homo sapiens mus musculus

SEQ ID NO: 153 - protein, 218 aa, Artificial; identical to SEQ ID NO: 144
  Chimeric homo sapiens mus musculus

SEQ ID NO: 154 - protein, 796 aa, Artificial
  Chimeric homo sapiens mus musculus
QVQLQQSGAELVRPGSSVKISCKASGYAFSSYWMNWVKQRPGQGLEWIGQIWPGDGDTNYNGKFKGKATLTADESSSTAYMQLSSLASEDSAVYFCARRETTTVGRYYYAMDYWGQGTTVTVSSASTKGPSVFPLAPSSKSTSGGTAALGCLVKDYFPEPVTVSWNSGALTSGVHTFPAVLQSSGLYSLSSVVTVPSSSLGTQTYICNVNHKPSNTKVDKRVEPKSCGGGSSAPELLGGPSVFLFPPKPKDTLMISRTPEVTCVVVDVSHEDPEVKFNWYVDGVEVHNAKTKPREEQYSSTYRVVSVLTVLHQDWLNGKEYKCKVSNKALPAPIEKTISKAKGQPREPQVYTLPPSREEMTKNQVSLTCLVKGFYPSDIAVEWESNGQPENNYKTTPPVLDSDGSFFLYSKLTVDKSRWQQGNVFSCSVMHEALHNHYTQKSLSLSPGGGGGSGGGGSGGGGSGQPREPQVYTLPPSREEMTKNQVSLTCLVKGFYPSDIAVEWESNGQPENNYKTTPPVLDSDGSFFLYSKLTVDKSRWQQGNVFSCSVMHEALHNHYTQKSLSLSPGSTGSEVQLQQSGPELVKPGASVKISCKTSGYTFTEYTMHWVKQSHGKSLEWIGGISPNIGGTSYNQKFKGKATLTVDKSSSTAYMELRSLTSEDSAVYYCARRGGSFDYWGQGTTLTVSSRTVAAPSVFIFPPSDEQLKSGTASVVCLLNNFYPREAKVQWKVDNALQSGNSQESVTEQDSKDSTYSLSSTLTLSKADYEKHKVYACEVTHQGLSSPVTKSFNRGEC

SEQ ID NO: 155 - protein, 214 aa, Artificial; identical to SEQ ID NO: 146
  Chimeric homo sapiens mus musculus

SEQ ID NO: 156 - protein, 218 aa, Artificial; identical to SEQ ID NO: 144
  Chimeric homo sapiens mus musculus

SEQ ID NO: 157 - protein, 819 aa, Artificial
  Chimeric homo sapiens mus musculus
QVQLQQSGAELVRPGSSVKISCKASGYAFSSYWMNWVKQRPGQGLEWIGQIWPGDGDTNYNGKFKGKATLTADESSSTAYMQLSSLASEDSAVYFCARRETTTVGRYYYAMDYWGQGTTVTVSSASTKGPSVFPLAPSSKSTSGGTAALGCLVKDYFPEPVTVSWNSGALTSGVHTFPAVLQSSGLYSLSSVVTVPSSSLGTQTYICNVNHKPSNTKVDKRVEPKSCDKTHTCPPCPAPELLGGPSVFLFPPKPKDTLMISRTPEVTCVVVDVSHEDPEVKFNWYVDGVEVHNAKTKPREEQYSSTYRVVSVLTVLHQDWLNGKEYKCKVSNKALPAPIEKTISKAKGQPREPQVYTLPPSREEMTKNQVSLTCLVKGFYPSDIAVEWESNGQPENNYKTTPPVLDSDGSFFLYSKLTVDKSRWQQGNVFSCSVMHEALHNHYTQKSLSLSPGGGGGSGGGGSGGGGSGQPREPQVYTLPPSREEMTKNQVSLTCLVKGFYPSDIAVEWESNGQPENNYKTTPPVLDSDGSFFLYSKLTVDKSRWQQGNVFSCSVMHEALHNHYTQKSLSLSPGSTGSEVQLQQSGPELVKPGASVKISCKTSGYTFTEYTMHWVKQSHGKSLEWIGGISPNIGGTSYNQKFKGKATLTVDKSSSTAYMELRSLTSEDSAVYYCARRGGSFDYWGQGTTLTVSSVEGGSGGSGGSGGSGGVDDIVMTQSPATLSVTPGDRVSLSCRASQSISDYLHWYQQKSHESPRLLIKYASQSISGIPSRFSGSGSGSDFTLSINSVEPEDVGVYYCQNGHSFPLTFGAGTKLELK

SEQ ID NO: 158 - protein, 218 aa, Artificial; identical to SEQ ID NO: 144
  Chimeric homo sapiens mus musculus

SEQ ID NO: 159 - protein, 819 aa, Artificial
  Chimeric homo sapiens mus musculus
QVQLQQSGAELVRPGSSVKISCKASGYAFSSYWMNWVKQRPGQGLEWIGQIWPGDGDTNYNGKFKGKATLTADESSSTAYMQLSSLASEDSAVYFCARRETTTVGRYYYAMDYWGQGTTVTVSSASTKGPSVFPLAPSSKSTSGGTAALGCLVKDYFPEPVTVSWNSGALTSGVHTFPAVLQSSGLYSLSSVVTVPSSSLGTQTYICNVNHKPSNTKVDKRVEPKSCDKTHTSPPSPAPELLGGPSVFLFPPKPKDTLMISRTPEVTCVVVDVSHEDPEVKFNWYVDGVEVHNAKTKPREEQYSSTYRVVSVLTVLHQDWLNGKEYKCKVSNKALPAPIEKTISKAKGQPREPQVYTLPPSREEMTKNQVSLTCLVKGFYPSDIAVEWESNGQPENNYKTTPPVLDSDGSFFLYSKLTVDKSRWQQGNVFSCSVMHEALHNHYTQKSLSLSPGGGGGSGGGGSGGGGSGQPREPQVYTLPPSREEMTKNQVSLTCLVKGFYPSDIAVEWESNGQPENNYKTTPPVLDSDGSFFLYSKLTVDKSRWQQGNVFSCSVMHEALHNHYTQKSLSLSPGSTGSEVQLQQSGPELVKPGASVKISCKTSGYTFTEYTMHWVKQSHGKSLEWIGGISPNIGGTSYNQKFKGKATLTVDKSSSTAYMELRSLTSEDSAVYYCARRGGSFDYWGQGTTLTVSSVEGGSGGSGGSGGSGGVDDIVMTQSPATLSVTPGDRVSLSCRASQSISDYLHWYQQKSHESPRLLIKYASQSISGIPSRFSGSGSGSDFTLSINSVEPEDVGVYYCQNGHSFPLTFGAGTKLELK

SEQ ID NO: 160 - protein, 218 aa, Artificial; identical to SEQ ID NO: 144
  Chimeric homo sapiens mus musculus

SEQ ID NO: 161 - protein, 815 aa, Artificial
  Chimeric homo sapiens mus musculus
QVQLQQSGAELVRPGSSVKISCKASGYAFSSYWMNWVKQRPGQGLEWIGQIWPGDGDTNYNGKFKGKATLTADESSSTAYMQLSSLASEDSAVYFCARRETTTVGRYYYAMDYWGQGTTVTVSSASTKGPSVFPLAPSSKSTSGGTAALGCLVKDYFPEPVTVSWNSGALTSGVHTFPAVLQSSGLYSLSSVVTVPSSSLGTQTYICNVNHKPSNTKVDKRVEPKSCGGGSSPAPELLGGPSVFLFPPKPKDTLMISRTPEVTCVVVDVSHEDPEVKFNWYVDGVEVHNAKTKPREEQYSSTYRVVSVLTVLHQDWLNGKEYKCKVSNKALPAPIEKTISKAKGQPREPQVYTLPPSREEMTKNQVSLTCLVKGFYPSDIAVEWESNGQPENNYKTTPPVLDSDGSFFLYSKLTVDKSRWQQGNVFSCSVMHEALHNHYTQKSLSLSPGGGGGSGGGGSGGGGSGQPREPQVYTLPPSREEMTKNQVSLTCLVKGFYPSDIAVEWESNGQPENNYKTTPPVLDSDGSFFLYSKLTVDKSRWQQGNVFSCSVMHEALHNHYTQKSLSLSPGSTGSEVQLQQSGPELVKPGASVKISCKTSGYTFTEYTMHWVKQSHGKSLEWIGGISPNIGGTSYNQKFKGKATLTVDKSSSTAYMELRSLTSEDSAVYYCARRGGSFDYWGQGTTLTVSSVEGGSGGSGGSGGSGGVDDIVMTQSPATLSVTPGDRVSLSCRASQSISDYLHWYQQKSHESPRLLIKYASQSISGIPSRFSGSGSGSDFTLSINSVEPEDVGVYYCQNGHSFPLTFGAGTKLELK

SEQ ID NO: 162 - protein, 819 aa, Artificial
  Chimeric homo sapiens mus musculus
DIQLTQSPASLAVSLGQRATISCKASQSVDYDGDSYLNWYQQIPGQPPKLLIYDASNLVSGIPPRFSGSGSGTDFTLNIHPVEKVDAATYHCQQSTEDPWTFGGGTKLEIKGGGGSGGGGSGGGGSQVQLQQSGAELVRPGSSVKISCKASGYAFSSYWMNWVKQRPGQGLEWIGQIWPGDGDTNYNGKFKGKATLTADESSSTAYMQLSSLASEDSAVYFCARRETTTVGRYYYAMDYWGQGTTVTVSSGGGSSAPELLGGPSVFLFPPKPKDTLMISRTPEVTCVVVDVSHEDPEVKFNWYVDGVEVHNAKTKPREEQYSSTYRVVSVLTVLHQDWLNGKEYKCKVSNKALPAPIEKTISKAKGQPREPQVYTLPPSREEMTKNQVSLTCLVKGFYPSDIAVEWESNGQPENNYKTTPPVLDSDGSFFLYSKLTVDKSRWQQGNVFSCSVMHEALHNHYTQKSLSLSPGGGGGSGGGGSGGGGSGQPREPQVYTLPPSREEMTKNQVSLTCLVKGFYPSDIAVEWESNGQPENNYKTTPPVLDSDGSFFLYSKLTVDKSRWQQGNVFSCSVMHEALHNHYTQKSLSLSPGSTGSEVQLQQSGPELVKPGASVKISCKTSGYTFTEYTMHWVKQSHGKSLEWIGGISPNIGGTSYNQKFKGKATLTVDKSSSTAYMELRSLTSEDSAVYYCARRGGSFDYWGQGTTLTVSSRTVAAPSVFIFPPSDEQLKSGTASVVCLLNNFYPREAKVQWKVDNALQSGNSQESVTEQDSKDSTYSLSSTLTLSKADYEKHKVYACEVTHQGLSSPVTKSFNRGEC

SEQ ID NO: 163 - protein, 214 aa, Artificial; identical to SEQ ID NO: 146
  Chimeric homo sapiens mus musculus

SEQ ID NO: 164 - protein, 819 aa, Artificial
  Chimeric homo sapiens mus musculus
DIQLTQSPASLAVSLGQRATISCKASQSVDYDGDSYLNWYQQIPGQPPKLLIYDASNLVSGIPPRFSGSGSGTDFTLNIHPVEKVDAATYHCQQSTEDPWTFGGGTKLEIKGGGGSGGGGSGGGGSQVQLQQSGAELVRPGSSVKISCKASGYAFSSYWMNWVKQRPGQGLEWIGQIWPGDGDTNYNGKFKGKATLTADESSSTAYMQLSSLASEDSAVYFCARRETTTVGRYYYAMDYWGQGTTVTVSSGGGSSAPELLGGPSVFLFPPKPKDTLMISRTPEVTCVVVDVSHEDPEVKFNWYVDGVEVHNAKTKPREEQYSSTYRVVSVLTVLHQDWLNGKEYKCKVSNKALPAPIEKTISKAKGQPREPQVYTLPPSREEMTKNQVSLTCLVKGFYPSDIAVEWESNGQPENNYKTTPPVLDSDGSFFLYSKLTVDKSRWQQGNVFSCSVMHEALHNHYTQKSLSLSPGGGGGSGGGGSGGGGSGQPREPQVYTLPPSREEMTKNQVSLTCLVKGFYPSDIAVEWESNGQPENNYKTTPPVLDSDGSFFLYSKLTVDKSRWQQGNVFSCSVMHEALHNHYTQKSLSLSPGSTGSEVQLQQSGPELVKPGASVKISCKTSGYTFTEYTMHWVKQSHGKSLEWIGGISPNIGGTSYNQKFKGKATLTVDKSSSTAYMELRSLTSEDSAVYYCARRGGSFDYWGQGTTLTVSSASTKGPSVFPLAPSSKSTSGGTAALGCLVKDYFPEPVTVSWNSGALTSGVHTFPAVLQSSGLYSLSSVVTVPSSSLGTQTYICNVNHKPSNTKVDKRVEPKSCDKTH

SEQ ID NO: 165 - protein, 214 aa, Artificial; identical to SEQ ID NO: 141
  Chimeric homo sapiens mus musculus

SEQ ID NO: 166 - protein, 218 aa, Artificial; identical to SEQ ID NO: 144
  Chimeric homo sapiens mus musculus

SEQ ID NO: 167 - protein, 792 aa, Artificial
  Chimeric homo sapiens mus musculus
QVQLQQSGAELVRPGSSVKISCKASGYAFSSYWMNWVKQRPGQGLEWIGQIWPGDGDTNYNGKFKGKATLTADESSSTAYMQLSSLASEDSAVYFCARRETTTVGRYYYAMDYWGQGTTVTVSSASTKGPSVFPLAPSSKSTSGGTAALGCLVKDYFPEPVTVSWNSGALTSGVHTFPAVLQSSGLYSLSSVVTVPSSSLGTQTYICNVNHKPSNTKVDKRVEPKSCDKTHTSPPSPAPELLGGPSVFLFPPKPKDTLMISRTPEVTCVVVDVSHEDPEVKFNWYVDGVEVHNAKTKPREEQYSSTYRVVSVLTVLHQDWLNGKEYKCKVSNKALPAPIEKTISKAKGQPREPQVYTLPPSREEMTKNQVSLTCLVKGFYPSDIAVEWESNGQPENNYKTTPPVLDSDGSFFLYSKLTVDKSRWQQGNVFSCSVMHEALHNHYTQKSLSLSPGGGGGSGGGGSGGGGSGQPREPQVYTLPPSREEMTKNQVSLTCLVKGFYPSDIAVEWESNGQPENNYKTTPPVLDSDGSFFLYSKLTVDKSRWQQGNVFSCSVMHEALHNHYTQKSLSLSPGSTGSDIVMTQSPATLSVTPGDRVSLSCRASQSISDYLHWYQQKSHESPRLLIKYASQSISGIPSRFSGSGSGSDFTLSINSVEPEDVGVYYCQNGHSFPLTFGAGTKLELKASTKGPSVFPLAPSSKSTSGGTAALGCLVKDYFPEPVTVSWNSGALTSGVHTFPAVLQSSGLYSLSSVVTVPSSSLGTQTYICNVNHKPSNTKVDKRVEPKSCDKTH

SEQ ID NO: 168 - protein, 223 aa, Artificial
  Chimeric homo sapiens mus musculus
EVQLQQSGPELVKPGASVKISCKTSGYTFTEYTMHWVKQSHGKSLEWIGGISPNIGGTSYNQKFKGKATLTVDKSSSTAYMELRSLTSEDSAVYYCARRGGSFDYWGQGTTLTVSSRTVAAPSVFIFPPSDEQLKSGTASVVCLLNNFYPREAKVQWKVDNALQSGNSQESVTEQDSKDSTYSLSSTLTLSKADYEKHKVYACEVTHQGLSSPVTKSFNRGEC

SEQ ID NO: 169 - protein, 445 aa, Artificial
  Chimeric homo sapiens mus musculus
DIQLTQSPASLAVSLGQRATISCKASQSVDYDGDSYLNWYQQIPGQPPKLLIYDASNLVSGIPPRFSGSGSGTDFTLNIHPVEKVDAATYHCQQSTEDPWTFGGGTKLEIKRTVAAPSVFIFPPSDEQLKSGTASVVCLLNNFYPREAKVQWKVDNALQSGNSQESVTEQDSKDSTYSLSSTLTLSKADYEKHKVYACEVTHQGLSSPVTKSFNRGECDKTHTCPPCPAPELLGGPSVFLFPPKPKDTLMISRTPEVTCVVVDVSHEDPEVKFNWYVDGVEVHNAKTKPREEQYNSTYRVVSVLTVLHQDWLNGKEYKCKVSNKALPAPIEKTISKAKGQPREPQVYTLPPSREEMTKNQVSLTCLVKGFYPSDIAVEWESNGQPENNYKTTPPVLDSDGSFFLYSKLTVDKSRWQQGNVFSCSVMHEALHNHYTQKSLSLSPGK

SEQ ID NO: 170 - protein, 680 aa, Artificial
  Chimeric homo sapiens mus musculus
QVQLQQSGAELVRPGSSVKISCKASGYAFSSYWMNWVKQRPGQGLEWIGQIWPGDGDTNYNGKFKGKATLTADESSSTAYMQLSSLASEDSAVYFCARRETTTVGRYYYAMDYWGQGTTVTVSSASTKGPSVFPLAPSSKSTSGGTAALGCLVKDYFPEPVTVSWNSGALTSGVHTFPAVLQSSGLYSLSSVVTVPSSSLGTQTYICNVNHKPSNTKVDKRVEPKSCDKTHTCPPCPAPELLGGPSVFLFPPKPKDTLMISRTPEVTCVVVDVSHEDPEVKFNWYVDGVEVHNAKTKPREEQYNSTYRVVSVLTVLHQDWLNGKEYKCKVSNKALPAPIEKTISKAKGQPREPQVYTLPPSREEMTKNQVSLTCLVKGFYPSDIAVEWESNGQPENNYKTTPPVLDSDGSFFLYSKLTVDKSRWQQGNVFSCSVMHEALHNHYTQKSLSLSPGSTGSEVQLQQSGPELVKPGASVKISCKTSGYTFTEYTMHWVKQSHGKSLEWIGGISPNIGGTSYNQKFKGKATLTVDKSSSTAYMELRSLTSEDSAVYYCARRGGSFDYWGQGTTLTVSSRTVAAPSVFIFPPSDEQLKSGTASVVCLLNNFYPREAKVQWKVDNALQSGNSQESVTEQDSKDSTYSLSSTLTLSKADYEKHKVYACEVTHQGLSSPVTKSFNRGEC

SEQ ID NO: 171 - protein, 214 aa, Artificial; identical to SEQ ID NO: 146
  Chimeric homo sapiens mus musculus

SEQ ID NO: 172 - protein, 445 aa, Artificial
  Chimeric homo sapiens mus musculus
DIQLTQSPASLAVSLGQRATISCKASQSVDYDGDSYLNWYQQIPGQPPKLLIYDASNLVSGIPPRFSGSGSGTDFTLNIHPVEKVDAATYHCQQSTEDPWTFGGGTKLEIKRTVAAPSVFIFPPSDEQLKSGTASVVCLLNNFYPREAKVQWKVDNALQSGNSQESVTEQDSKDSTYSLSSTLTLSKADYEKHKVYACEVTHQGLSSPVTKSFNRGECDKTHTCPPCPAPELLGGPSVFLFPPKPKDTLMISRTPEVTCVVVDVSHEDPEVKFNWYVDGVEVHNAKTKPREEQYSSTYRVVSVLTVLHQDWLNGKEYKCKVSNKALPAPIEKTISKAKGQPREPQVYTLPPSREEMTKNQVSLTCLVKGFYPSDIAVEWESNGQPENNYKTTPPVLDSDGSFFLYSKLTVDKSRWQQGNVFSCSVMHEALHNHYTQKSLSLSPGK

SEQ ID NO: 173 - protein, 680 aa, Artificial
  Chimeric homo sapiens mus musculus
QVQLQQSGAELVRPGSSVKISCKASGYAFSSYWMNWVKQRPGQGLEWIGQIWPGDGDTNYNGKFKGKATLTADESSSTAYMQLSSLASEDSAVYFCARRETTTVGRYYYAMDYWGQGTTVTVSSASTKGPSVFPLAPSSKSTSGGTAALGCLVKDYFPEPVTVSWNSGALTSGVHTFPAVLQSSGLYSLSSVVTVPSSSLGTQTYICNVNHKPSNTKVDKRVEPKSCDKTHTCPPCPAPELLGGPSVFLFPPKPKDTLMISRTPEVTCVVVDVSHEDPEVKFNWYVDGVEVHNAKTKPREEQYSSTYRVVSVLTVLHQDWLNGKEYKCKVSNKALPAPIEKTISKAKGQPREPQVYTLPPSREEMTKNQVSLTCLVKGFYPSDIAVEWESNGQPENNYKTTPPVLDSDGSFFLYSKLTVDKSRWQQGNVFSCSVMHEALHNHYTQKSLSLSPGSTGSEVQLQQSGPELVKPGASVKISCKTSGYTFTEYTMHWVKQSHGKSLEWIGGISPNIGGTSYNQKFKGKATLTVDKSSSTAYMELRSLTSEDSAVYYCARRGGSFDYWGQGTTLTVSSRTVAAPSVFIFPPSDEQLKSGTASVVCLLNNFYPREAKVQWKVDNALQSGNSQESVTEQDSKDSTYSLSSTLTLSKADYEKHKVYACEVTHQGLSSPVTKSFNRGEC

SEQ ID NO: 174 - protein, 214 aa, Artificial; identical to SEQ ID NO: 146
  Chimeric homo sapiens mus musculus

SEQ ID NO: 175 - protein, 445 aa, Artificial
  Chimeric homo sapiens mus musculus
DIQLTQSPASLAVSLGQRATISCKASQSVDYDGDSYLNWYQQIPGQPPKLLIYDASNLVSGIPPRFSGSGSGTDFTLNIHPVEKVDAATYHCQQSTEDPWTFGGGTKLEIKRTVAAPSVFIFPPSDEQLKSGTASVVCLLNNFYPREAKVQWKVDNALQSGNSQESVTEQDSKDSTYSLSSTLTLSKADYEKHKVYACEVTHQGLSSPVTKSFNRGESDKTHTCPPCPAPELLGGPSVFLFPPKPKDTLMISRTPEVTCVVVDVSHEDPEVKFNWYVDGVEVHNAKTKPREEQYSSTYRVVSVLTVLHQDWLNGKEYKCKVSNKALPAPIEKTISKAKGQPREPQVYTLPPSREEMTKNQVSLTCLVKGFYPSDIAVEWESNGQPENNYKTTPPVLDSDGSFFLYSKLTVDKSRWQQGNVFSCSVMHEALHNHYTQKSLSLSPGK

SEQ ID NO: 176 - protein, 680 aa, Artificial
  Chimeric homo sapiens mus musculus
QVQLQQSGAELVRPGSSVKISCKASGYAFSSYWMNWVKQRPGQGLEWIGQIWPGDGDTNYNGKFKGKATLTADESSSTAYMQLSSLASEDSAVYFCARRETTTVGRYYYAMDYWGQGTTVTVSSASTKGPSVFPLAPSSKSTSGGTAALGCLVKDYFPEPVTVSWNSGALTSGVHTFPAVLQSSGLYSLSSVVTVPSSSLGTQTYICNVNHKPSNTKVDKRVEPKSSDKTHTCPPCPAPELLGGPSVFLFPPKPKDTLMISRTPEVTCVVVDVSHEDPEVKFNWYVDGVEVHNAKTKPREEQYSSTYRVVSVLTVLHQDWLNGKEYKCKVSNKALPAPIEKTISKAKGQPREPQVYTLPPSREEMTKNQVSLTCLVKGFYPSDIAVEWESNGQPENNYKTTPPVLDSDGSFFLYSKLTVDKSRWQQGNVFSCSVMHEALHNHYTQKSLSLSPGSTGSEVQLQQSGPELVKPGASVKISCKTSGYTFTEYTMHWVKQSHGKSLEWIGGISPNIGGTSYNQKFKGKATLTVDKSSSTAYMELRSLTSEDSAVYYCARRGGSFDYWGQGTTLTVSSRTVAAPSVFIFPPSDEQLKSGTASVVCLLNNFYPREAKVQWKVDNALQSGNSQESVTEQDSKDSTYSLSSTLTLSKADYEKHKVYACEVTHQGLSSPVTKSFNRGEC

SEQ ID NO: 177 - protein, 214 aa, Artificial; identical to SEQ ID NO: 146
  Chimeric homo sapiens mus musculus

SEQ ID NO: 178 - protein, 445 aa, Artificial; identical to SEQ ID NO: 169
  Chimeric homo sapiens mus musculus

SEQ ID NO: 179 - protein, 698 aa, Artificial
  Chimeric homo sapiens mus musculus
QVQLQQSGAELVRPGSSVKISCKASGYAFSSYWMNWVKQRPGQGLEWIGQIWPGDGDTNYNGKFKGKATLTADESSSTAYMQLSSLASEDSAVYFCARRETTTVGRYYYAMDYWGQGTTVTVSSASTKGPSVFPLAPSSKSTSGGTAALGCLVKDYFPEPVTVSWNSGALTSGVHTFPAVLQSSGLYSLSSVVTVPSSSLGTQTYICNVNHKPSNTKVDKRVEPKSCDKTHTCPPCPAPELLGGPSVFLFPPKPKDTLMISRTPEVTCVVVDVSHEDPEVKFNWYVDGVEVHNAKTKPREEQYNSTYRVVSVLTVLHQDWLNGKEYKCKVSNKALPAPIEKTISKAKGQPREPQVYTLPPSREEMTKNQVSLTCLVKGFYPSDIAVEWESNGQPENNYKTTPPVLDSDGSFFLYSKLTVDKSRWQQGNVFSCSVMHEALHNHYTQKSLSLSPGSTGSEVQLQQSGPELVKPGASVKISCKTSGYTFTEYTMHWVKQSHGKSLEWIGGISPNIGGTSYNQKFKGKATLTVDKSSSTAYMELRSLTSEDSAVYYCARRGGSFDYWGQGTTLTVSSVEGGSGGSGGSGGSGGVDDIVMTQSPATLSVTPGDRVSLSCRASQSISDYLHWYQQKSHESPRLLIKYASQSISGIPSRFSGSGSGSDFTLSINSVEPEDVGVYYCQNGHSFPLTFGAGTKLELK

SEQ ID NO: 180 - protein, 445 aa, Artificial; identical to SEQ ID NO: 172
  Chimeric homo sapiens mus musculus

SEQ ID NO: 181 - protein, 698 aa, Artificial
  Chimeric homo sapiens mus musculus
QVQLQQSGAELVRPGSSVKISCKASGYAFSSYWMNWVKQRPGQGLEWIGQIWPGDGDTNYNGKFKGKATLTADESSSTAYMQLSSLASEDSAVYFCARRETTTVGRYYYAMDYWGQGTTVTVSSASTKGPSVFPLAPSSKSTSGGTAALGCLVKDYFPEPVTVSWNSGALTSGVHTFPAVLQSSGLYSLSSVVTVPSSSLGTQTYICNVNHKPSNTKVDKRVEPKSCDKTHTCPPCPAPELLGGPSVFLFPPKPKDTLMISRTPEVTCVVVDVSHEDPEVKFNWYVDGVEVHNAKTKPREEQYSSTYRVVSVLTVLHQDWLNGKEYKCKVSNKALPAPIEKTISKAKGQPREPQVYTLPPSREEMTKNQVSLTCLVKGFYPSDIAVEWESNGQPENNYKTTPPVLDSDGSFFLYSKLTVDKSRWQQGNVFSCSVMHEALHNHYTQKSLSLSPGSTGSEVQLQQSGPELVKPGASVKISCKTSGYTFTEYTMHWVKQSHGKSLEWIGGISPNIGGTSYNQKFKGKATLTVDKSSSTAYMELRSLTSEDSAVYYCARRGGSFDYWGQGTTLTVSSVEGGSGGSGGSGGSGGVDDIVMTQSPATLSVTPGDRVSLSCRASQSISDYLHWYQQKSHESPRLLIKYASQSISGIPSRFSGSGSGSDFTLSINSVEPEDVGVYYCQNGHSFPLTFGAGTKLELK

SEQ ID NO: 182 - protein, 454 aa, Artificial
  Chimeric homo sapiens mus musculus
QVQLQQSGAELVRPGSSVKISCKASGYAFSSYWMNWVKQRPGQGLEWIGQIWPGDGDTNYNGKFKGKATLTADESSSTAYMQLSSLASEDSAVYFCARRETTTVGRYYYAMDYWGQGTTVTVSSASTKGPSVFPLAPSSKSTSGGTAALGCLVKDYFPEPVTVSWNSGALTSGVHTFPAVLQSSGLYSLSSVVTVPSSSLGTQTYICNVNHKPSNTKVDKRVEPKSCDKTHTCPPCPAPELLGGPSVFLFPPKPKDTLMISRTPEVTCVVVDVSHEDPEVKFNWYVDGVEVHNAKTKPREEQYSSTYRVVSVLTVLHQDWLNGKEYKCKVSNKALPAPIEKTISKAKGQPREPQVYTLPPSREEMTKNQVSLTCLVKGFYPSDIAVEWESNGQPENNYKTTPPVLDSDGSFFLYSKLTVDKSRWQQGNVFSCSVMHEALHNHYTQKSLSLSPGK

SEQ ID NO: 183 - protein, 670 aa, Artificial
  Chimeric homo sapiens mus musculus
DIQLTQSPASLAVSLGQRATISCKASQSVDYDGDSYLNWYQQIPGQPPKLLIYDASNLVSGIPPRFSGSGSGTDFTLNIHPVEKVDAATYHCQQSTEDPWTFGGGTKLEIKRTVAAPSVFIFPPSDEQLKSGTASVVCLLNNFYPREAKVQWKVDNALQSGNSQESVTEQDSKDSTYSLSSTLTLSKADYEKHKVYACEVTHQGLSSPVTKSFNRGECDKTHTCPPCPAPELLGGPSVFLFPPKPKDTLMISRTPEVTCVVVDVSHEDPEVKFNWYVDGVEVHNAKTKPREEQSSTYRVVSVLTVLHQDWLNGKEYKCKVSNKALPAPIEKTISKAKGQPREPQVYTLPPSREEMTKNQVSLTCLVKGFYPSDIAVEWESNGQPENNYKTTPPVLDSDGSFFLYSKLTVDKSRWQQGNVFSCSVMHEALHNHYTQKSLSLSPGSTGSEVQLQQSGPELVKPGASVKISCKTSGYTFTEYTMHWVKQSHGKSLEWIGGISPNIGGTSYNQKFKGKATLTVDKSSSTAYMELRSLTSEDSAVYYCARRGGSFDYWGQGTTLTVSSRTVAAPSVFIFPPSDEQLKSGTASVVCLLNNFYPREAKVQWKVDNALQSGNSQESVTEQDSKDSTYSLSSTLTLSKADYEKHKVYACEVTHQGLSSPVTKSFNRGEC

SEQ ID NO: 184 - protein, 214 aa, Artificial; identical to SEQ ID NO: 146
  Chimeric homo sapiens mus musculus

SEQ ID NO: 185 - protein, 445 aa, Artificial; identical to SEQ ID NO: 172
  Chimeric homo sapiens mus musculus

SEQ ID NO: 186 - protein, 671 aa, Artificial
  Chimeric homo sapiens mus musculus
QVQLQQSGAELVRPGSSVKISCKASGYAFSSYWMNWVKQRPGQGLEWIGQIWPGDGDTNYNGKFKGKATLTADESSSTAYMQLSSLASEDSAVYFCARRETTTVGRYYYAMDYWGQGTTVTVSSASTKGPSVFPLAPSSKSTSGGTAALGCLVKDYFPEPVTVSWNSGALTSGVHTFPAVLQSSGLYSLSSVVTVPSSSLGTQTYICNVNHKPSNTKVDKRVEPKSCDKTHTCPPCPAPELLGGPSVFLFPPKPKDTLMISRTPEVTCVVVDVSHEDPEVKFNWYVDGVEVHNAKTKPREEQYSSTYRVVSVLTVLHQDWLNGKEYKCKVSNKALPAPIEKTISKAKGQPREPQVYTLPPSREEMTKNQVSLTCLVKGFYPSDIAVEWESNGQPENNYKTTPPVLDSDGSFFLYSKLTVDKSRWQQGNVFSCSVMHEALHNHYTQKSLSLSPGSTGSDIVMTQSPATLSVTPGDRVSLSCRASQSISDYLHWYQQKSHESPRLLIKYASQSISGIPSRFSGSGSGSDFTLSINSVEPEDVGVYYCQNGHSFPLTFGAGTKLELKASTKGPSVFPLAPSSKSTSGGTAALGCLVKDYFPEPVTVSWNSGALTSGVHTFPAVLQSSGLYSLSSVVTVPSSSLGTQTYICNVNHKPSNTKVDKRVEPKSCDKTH

SEQ ID NO: 187 - protein, 223 aa, Artificial; identical to SEQ ID NO: 168
  Chimeric homo sapiens mus musculus

SEQ ID NO: 188 - protein, 680 aa, Artificial
  Human-mouse chimeric
QVQLVQSGAEVKKPGSSVKVSCKASGYAFSYSWINWVRQAPGQGLEWMGRIFPGDGDTDYNGKFKGRVTITADKSTSTAYMELSSLRSEDTAVYYCARNVFDGYWLVYWGQGTLVTVSSASTKGPSVFPLAPSSKSTSGGTAALGCLVKDYFPEPVTVSWNSGALTSGVHTFPAVLQSSGLYSLSSVVTVPSSSLGTQTYICNVNHKPSNTKVDKRVEPKSCDKTHTCPPCPAPELLGGPSVFLFPPKPKDTLMISRTPEVTCVVVDVSHEDPEVKFNWYVDGVEVHNAKTKPREEQYNSTYRVVSVLTVLHQDWLNGKEYKCKVSNKALPAPIEKTISKAKGQPREPQVYTLPPSREEMTKNQVSLTCLVKGFYPSDIAVEWESNGQPENNYKTTPPVLDSDGSFFLYSKLTVDKSRWQQGNVFSCSVMHEALHNHYTQKSLSLSPGSTGSQVQLQQPGAELVKPGASVKMSCKASGYTFTSYNMHWVKQTPGRGLEWIGAIYPGNGDTSYNQKFKGKATLTADKSSSTAYMQLSSLTSEDSAVYYCARSTYYGGDWYFNVWGAGTTVTVSARTVAAPSVFIFPPSDEQLKSGTASVVCLLNNFYPREAKVQWKVDNALQSGNSQESVTEQDSKDSTYSLSSTLTLSKADYEKHKVYACEVTHQGLSSPVTKSFNRGEC

SEQ ID NO: 189 - protein, 446 aa, Artificial
  Human-mouse chimeric
DIVMTQTPLSLPVTPGEPASISCRSSKSLLHSNGITYLYWYLQKPGQSPQLLIYQMSNLVSGVPDRFSGSGSGTDFTLKISRVEAEDVGVYYCAQNLELPYTFGGGTKVEIKRTVAAPSVFIFPPSDEQLKSGTASVVCLLNNFYPREAKVQWKVDNALQSGNSQESVTEQDSKDSTYSLSSTLTLSKADYEKHKVYACEVTHQGLSSPVTKSFNRGECDKTHTCPPCPAPELLGGPSVFLFPPKPKDTLMISRTPEVTCVVVDVSHEDPEVKFNWYVDGVEVHNAKTKPREEQYNSTYRVVSVLTVLHQDWLNGKEYKCKVSNKALPAPIEKTISKAKGQPREPQVYTLPPSREEMTKNQVSLTCLVKGFYPSDIAVEWESNGQPENNYKTTPPVLDSDGSFFLYSKLTVDKSRWQQGNVFSCSVMHEALHNHYTQKSLSLSPGK

SEQ ID NO: 190 - protein, 459 aa, Artificial
  Human-mouse chimeric
QIVLSQSPAILSASPGEKVTMTCRASSSVSYIHWFQQKPGSSPKPWIYATSNLASGVPVRFSGSGSGTSYSLTISRVEAEDAATYYCQQWTSNPPTFGGGTKLEIKASTKGPSVFPLAPSSKSTSGGTAALGCLVKDYFPEPVTVSWNSGALTSGVHTFPAVLQSSGLYSLSSVVTVPSSSLGTQTYICNVNHKPSNTKVDKRVEPKSCDKTHGGSSSEVQLQQSGPELVKPGASVKISCKTSGYTFTEYTMHWVKQSHGKSLEWIGGISPNIGGTSYNQKFKGKATLTVDKSSSTAYMELRSLTSEDSAVYYCARRGGSFDYWGQGTTLTVSSVEGGSGGSGGSGGSGGVDDIVMTQSPATLSVTPGDRVSLSCRASQSISDYLHWYQQKSHESPRLLIKYASQSISGIPSRFSGSGSGSDFTLSINSVEPEDVGVYYCQNGHSFPLTFGAGTKLELK

SEQ ID NO: 191 - protein, 446 aa, Artificial
  Human-mouse chimeric
DIVMTQTPLSLPVTPGEPASISCRSSKSLLHSNGITYLYWYLQKPGQSPQLLIYQMSNLVSGVPDRFSGSGSGTDFTLKISRVEAEDVGVYYCAQNLELPYTFGGGTKVEIKRTVAAPSVFIFPPSDEQLKSGTASVVCLLNNFYPREAKVQWKVDNALQSGNSQESVTEQDSKDSTYSLSSTLTLSKADYEKHKVYACEVTHQGLSSPVTKSFNRGECDKTHTCPPCPAPELLGGPSVFLFPPKPKDTLMISRTPEVTCVVVDVSHEDPEVKFNWYVDGVEVHNAKTKPREEQYSSTYRVVSVLTVLHQDWLNGKEYKCKVSNKALPAPIEKTISKAKGQPREPQVYTLPPSREEMTKNQVSLTCLVKGFYPSDIAVEWESNGQPENNYKTTPPVLDSDGSFFLYSKLTVDKSRWQQGNVFSCSVMHEALHNHYTQKSLSLSPGK

SEQ ID NO: 192 - protein, 680 aa, Artificial
  Human mouse chimeric
QVQLVQSGAEVKKPGSSVKVSCKASGYAFSYSWINWVRQAPGQGLEWMGRIFPGDGDTDYNGKFKGRVTITADKSTSTAYMELSSLRSEDTAVYYCARNVFDGYWLVYWGQGTLVTVSSASTKGPSVFPLAPSSKSTSGGTAALGCLVKDYFPEPVTVSWNSGALTSGVHTFPAVLQSSGLYSLSSVVTVPSSSLGTQTYICNVNHKPSNTKVDKRVEPKSCDKTHTCPPCPAPELLGGPSVFLFPPKPKDTLMISRTPEVTCVVVDVSHEDPEVKFNWYVDGVEVHNAKTKPREEQYSSTYRVVSVLTVLHQDWLNGKEYKCKVSNKALPAPIEKTISKAKGQPREPQVYTLPPSREEMTKNQVSLTCLVKGFYPSDIAVEWESNGQPENNYKTTPPVLDSDGSFFLYSKLTVDKSRWQQGNVFSCSVMHEALHNHYTQKSLSLSPGSTGSQVQLQQPGAELVKPGASVKMSCKASGYTFTSYNMHWVKQTPGRGLEWIGAIYPGNGDTSYNQKFKGKATLTADKSSSTAYMQLSSLTSEDSAVYYCARSTYYGGDWYFNVWGAGTTVTVSARTVAAPSVFIFPPSDEQLKSGTASVVCLLNNFYPREAKVQWKVDNALQSGNSQESVTEQDSKDSTYSLSSTLTLSKADYEKHKVYACEVTHQGLSSPVTKSFNRGEC

SEQ ID NO: 193 - protein, 459 aa, Artificial; identical to SEQ ID NO: 190
  Human mouse chimeric

SEQ ID NO: 194 - protein, 801 aa, Artificial
  Human-mouse chimeric
QVQLVQSGAEVKKPGSSVKVSCKASGYAFSYSWINWVRQAPGQGLEWMGRIFPGDGDTDYNGKFKGRVTITADKSTSTAYMELSSLRSEDTAVYYCARNVFDGYWLVYWGQGTLVTVSSASTKGPSVFPLAPSSKSTSGGTAALGCLVKDYFPEPVTVSWNSGALTSGVHTFPAVLQSSGLYSLSSVVTVPSSSLGTQTYICNVNHKPSNTKVDKRVEPKSCDKTHTSPPSPAPELLGGPSVFLFPPKPKDTLMISRTPEVTCVVVDVSHEDPEVKFNWYVDGVEVHNAKTKPREEQYSSTYRVVSVLTVLHQDWLNGKEYKCKVSNKALPAPIEKTISKAKGQPREPQVYTLPPSREEMTKNQVSLTCLVKGFYPSDIAVEWESNGQPENNYKTTPPVLDSDGSFFLYSKLTVDKSRWQQGNVFSCSVMHEALHNHYTQKSLSLSPGGGGGSGGGGSGGGGSGQPREPQVYTLPPSREEMTKNQVSLTCLVKGFYPSDIAVEWESNGQPENNYKTTPPVLDSDGSFFLYSKLTVDKSRWQQGNVFSCSVMHEALHNHYTQKSLSLSPGSTGSQVQLQQPGAELVKPGASVKMSCKASGYTFTSYNMHWVKQTPGRGLEWIGAIYPGNGDTSYNQKFKGKATLTADKSSSTAYMQLSSLTSEDSAVYYCARSTYYGGDWYFNVWGAGTTVTVSARTVAAPSVFIFPPSDEQLKSGTASVVCLLNNFYPREAKVQWKVDNALQSGNSQESVTEQDSKDSTYSLSSTLTLSKADYEKHKVYACEVTHQGLSSPVTKSFNRGEC

SEQ ID NO: 195 - protein, 219 aa, Artificial
  Human-mouse chimeric
DIVMTQTPLSLPVTPGEPASISCRSSKSLLHSNGITYLYWYLQKPGQSPQLLIYQMSNLVSGVPDRFSGSGSGTDFTLKISRVEAEDVGVYYCAQNLELPYTFGGGTKVEIKRTVAAPSVFIFPPSDEQLKSGTASVVCLLNNFYPREAKVQWKVDNALQSGNSQESVTEQDSKDSTYSLSSTLTLSKADYEKHKVYACEVTHQGLSSPVTKSFNRGEC

SEQ ID NO: 196 - protein, 459 aa, Artificial; identical to SEQ ID NO: 190
  Human - mouse chimeric

SEQ ID NO: 197 - protein, 928 aa, Artificial
  Human-mouse chimeric
DIVMTQTPLSLPVTPGEPASISCRSSKSLLHSNGITYLYWYLQKPGQSPQLLIYQMSNLVSGVPDRFSGSGSGTDFTLKISRVEAEDVGVYYCAQNLELPYTFGGGTKVEIKGGGGSGGGGSGGGGSQVQLVQSGAEVKKPGSSVKVSCKASGYAFSYSWINWVRQAPGQGLEWMGRIFPGDGDTDYNGKFKGRVTITADKSTSTAYMELSSLRSEDTAVYYCARNVFDGYWLVYWGQGTLVTVSSASTKGPSVFPLAPSSKSTSGGTAALGCLVKDYFPEPVTVSWNSGALTSGVHTFPAVLQSSGLYSLSSVVTVPSSSLGTQTYICNVNHKPSNTKVDKRVEPKSCDKTHTSPPSPAPELLGGPSVFLFPPKPKDTLMISRTPEVTCVVVDVSHEDPEVKFNWYVDGVEVHNAKTKPREEQYSSTYRVVSVLTVLHQDWLNGKEYKCKVSNKALPAPIEKTISKAKGQPREPQVYTLPPSREEMTKNQVSLTCLVKGFYPSDIAVEWESNGQPENNYKTTPPVLDSDGSFFLYSKLTVDKSRWQQGNVFSCSVMHEALHNHYTQKSLSLSPGGGGGSGGGGSGGGGSGQPREPQVYTLPPSREEMTKNQVSLTCLVKGFYPSDIAVEWESNGQPENNYKTTPPVLDSDGSFFLYSKLTVDKSRWQQGNVFSCSVMHEALHNHYTQKSLSLSPGSTGSQVQLQQPGAELVKPGASVKMSCKASGYTFTSYNMHWVKQTPGRGLEWIGAIYPGNGDTSYNQKFKGKATLTADKSSSTAYMQLSSLTSEDSAVYYCARSTYYGGDWYFNVWGAGTTVTVSARTVAAPSVFIFPPSDEQLKSGTASVVCLLNNFYPREAKVQWKVDNALQSGNSQESVTEQDSKDSTYSLSSTLTLSKADYEKHKVYACEVTHQGLSSPVTKSFNRGEC

SEQ ID NO: 198 - protein, 459 aa, Artificial; identical to SEQ ID NO: 190
  Human - mouse chimeric

SEQ ID NO: 199 - protein, 120 aa, Artificial
  Chimeric
QVQLVQSGAEVKKPGSSVKVSCKASGYTFSDYVINWVRQAPGQGLEWMGEIYPGSGTNYYNEKFKAKATITADKSTSTAYMELSSLRSEDTAVYYCARRGRYGLYAMDYWGQGTTVTVSS

SEQ ID NO: 200 - protein, 120 aa, Artificial
  Chimeric
QVQLVQSGAEVKKPGSSVKVSCKASGYTFTDYVINWGRQAPGQGLEWIGEIYPGSGTNYYNEKFKAKATITADKSTSTAYMELSSLRSEDTAVYFCARRGRYGLYAMDYWGQGTTVTVSS

SEQ ID NO: 201 - protein, 107 aa, Artificial
  Chimeric
DIQMTQSPSSLSASVGDRVTITCRASQDISNYLNWYQQKPGKAPKLLIYYTSRLHSGVPSRFSGSGSGTDFTFTISSLQPEDIATYFCQQGNTRPWTFGGGTKVEIK

SEQ ID NO: 202 - protein, 122 aa, Artificial
  Chimeric
QVQLQESGPGLVKPSQTLSLTCTVSGYSISSDYAWNWIRQPPGKGLEWIGYITYSGSTSYNPSLESRVTISRDTSKNQFSLKLSSVTAADTAVYYCARGGYYGSSWGVFAYWGQGTLVTVSS

SEQ ID NO: 203 - protein, 122 aa, Artificial
  Chimeric
QVQLQESGPGLVKPSQTLSLTCTVSGYSISSDYAWNWIRQPPGKGLEWMGYITYSGSTSYNPSLESRITISRDTSKNQFSLKLSSVTAADTAVYYCARGGYYGSSWGVFAYWGQGTLVTVSS

SEQ ID NO: 204 - protein, 122 aa, Artificial
  Chimeric
QVQLQESGPGLVKPSQTLSLTCTVSGYSITSDYAWNWIRQPPGKGLEWMGYITYSGSTSYNPSLESRITISRDTSKNQFSLKLSSVTAADTAVYYCARGGYYGSSWGVFAYWGQGTLVTVSS

SEQ ID NO: 205 - protein, 107 aa, Artificial
  Chimeric
DIQMTQSPSSLSASVGDRVTITCRVSENIYSYLAWYQQKPGKAPKLLVYNAKTLAEGVPSRFSGSGSGTDFTLTISSLQPEDFATYYCQHHYGTPWTFGGGTKVEIK

SEQ ID NO: 206 - protein, 116 aa, Artificial
  Chimeric
QVQLVQSGAEVKKPGSSVKVSCKASGYTFSEYTMHWVRQAPGQGLEWMGGISPNIGGTSYNQKFKGRVTITADKSTSTAYMELSSLRSEDTAVYYCARRGGSFDYWGQGTTVTVSS

SEQ ID NO: 207 - protein, 116 aa, Artificial
  Chimeric
QVQLVQSGAEVKKPGSSVKVSCKASGYTFSEYTMHWVRQAPGQGLEWIGGISPNIGGTSYNQKFKGRATITADKSTSTAYMELSSLRSEDTAVYYCARRGGSFDYWGQGTTVTVSS

SEQ ID NO: 208 - protein, 116 aa, Artificial
  Chimeric
QVQLVQSGAEVKKPGSSVKVSCKASGYTFSEYTMHWVRQAPGQGLEWIGGISPNIGGTSYNQKFKGRATLTADKSTSTAYMELSSLRSEDTAVYYCARRGGSFDYWGQGTTVTVSS

SEQ ID NO: 209 - protein, 107 aa, Artificial
  Chimeric
EIVMTQSPATLSVSPGERATLSCRASQSISDYLHWYQQKPGQAPRLLIKYASQSISGIPARFSGSGSGTDFTLTISSLEPEDFAVYYCQNGHSFPLTFGQGTKLEIK

SEQ ID NO: 210 - protein, 117 aa, Artificial
  Chimeric
QVQLVQSGAEVKKPGASVKVSCKASGYTFTSFTMHWVRQAPGQGLEWIGYINPSSGYTEYNQKFKDRVTITADKSTSTAYMELSSLRSEDTAVYYCVRGSSRGFDYWGQGTLVTVSS

SEQ ID NO: 211 - protein, 117 aa, Artificial
  Chimeric
QVQLVQSGAEVKKPGASVKVSCKASGYTFTSFTMHWVRQAPGQGLEWIGYINPSSGYTEYNQKFKDRTTITADKSTSTAYMELSSLRSEDTAVYYCVRGSSRGFDYWGQGTLVTVSS

SEQ ID NO: 212 - protein, 117 aa, Artificial
  Chimeric
QVQLVQSGAEVKKPGASVKVSCKASGYTFTSFTMHWVRQAPGQGLEWIGYINPSSGYTEYNQKFKDRTTLTADKSTSTAYMELSSLRSEDTAVYYCVRGSSRGFDYWGQGTLVTVSS

SEQ ID NO: 213 - protein, 107 aa, Artificial
  Chimeric
DIQMTQSPSSLSASVGDRVTITCRASENIYSNLAWFQQKPGKAPKLLVYAATNLADGVPSRFSGSGSGTDYTLTISSLQPEDFATYYCQHFWGTPRTFGGGTKVEIK

SEQ ID NO: 214 - protein, 120 aa, Artificial
  Chimeric
QVQLQESGPGLVKPSQTLSLTCTVSGGSISSDYAWNWIRQPPGKGLEWIGYITYSGSTNYNPSLKSRVTISRDTSKNQFSLKLSSVTAADTAVYYCARCWDYALYAMDCWGQGTTVTVSS

SEQ ID NO: 215 - protein, 120 aa, Artificial
  Chimeric
QVQLQESGPGLVKPSQTLSLTCTVSGYSISSDYAWNWIRQPPGKGLEWIGYITYSGSTNYNPSLKSRVTISRDTSKNQFSLKLSSVTAADTAVYYCARCWDYALYAMDCWGQGTTVTVSS

SEQ ID NO: 216 - protein, 120 aa, Artificial
  Chimeric
QVQLQESGPGLVKPSQTLSLTCTVSGYSISSDYAWNWIRQPPGKGLEWMGYITYSGSTNYNPSLKSRITISRDTSKNQFSLKLSSVTAADTAVYYCARCWDYALYAMDCWGQGTTVTVSS

SEQ ID NO: 217 - protein, 107 aa, Artificial
  Chimeric
DIQMTQSPSSLSASVGDRVTITCRTSENIYSYLAWCQQKPGKAPKLLIYNAKTLAEGVPSRFSGSGSGTDFTLTISSLQPEDFATYYCQHHYDTPLTFGQGTKLEIK

SEQ ID NO: 218 - protein, 107 aa, Artificial
  Chimeric
DIQMTQSPSSLSASVGDRVTITCRTSENIYSYLAWCQQKPGKAPKLLVYNAKTLAEGVPSRFSGSGSGTDFTLTISSLQPEDFATYYCQHHYDTPLTFGQGTKLEIK